European Patent Specification EP 3 394 620 B1, published May 22, 2024. Title: Bladder Cancer Biomarker Proteins. Applicant: Polyquant GmbH et al. The sequence listing filed with the application follows.

SEQUENCE LISTING (945 sequences)

SEQ ID NO: 1 - protein, 10 aa, Homo sapiens
EHVAHLLFLR

SEQ ID NO: 2 - protein, 15 aa, Homo sapiens
NWGLSFYADKPETTK

SEQ ID NO: 3 - protein, 9 aa, Homo sapiens
SDVMYTDWK

SEQ ID NO: 4 - protein, 14 aa, Homo sapiens
ITPNLAEFAFSLYR

SEQ ID NO: 5 - protein, 15 aa, Homo sapiens
LQHLENELTHDIITK

SEQ ID NO: 6 - protein, 10 aa, Homo sapiens
LSITGTYDLK

SEQ ID NO: 7 - protein, 18 aa, Homo sapiens
LYHSEAFTVNFGDTEEAK

SEQ ID NO: 8 - protein, 10 aa, Homo sapiens
SVLGQLGITK

SEQ ID NO: 9 - protein, 11 aa, Homo sapiens
ATWSGAVLAGR

SEQ ID NO: 10 - protein, 12 aa, Homo sapiens
HQFLLTGDTQGR

SEQ ID NO: 11 - protein, 10 aa, Homo sapiens
DLLLPQPDLR

SEQ ID NO: 12 - protein, 9 aa, Homo sapiens
GQTLLAVAK

SEQ ID NO: 13 - protein, 10 aa, Homo sapiens
VAAGAFQGLR

SEQ ID NO: 14 - protein, 13 aa, Homo sapiens
LVHVEEPHTETVR

SEQ ID NO: 15 - protein, 12 aa, Homo sapiens
NEDSLVFVQTDK

SEQ ID NO: 16 - protein, 10 aa, Homo sapiens
QGIPFFGQVR

SEQ ID NO: 17 - protein, 10 aa, Homo sapiens
DADPDTFFAK

SEQ ID NO: 18 - protein, 7 aa, Homo sapiens
FTFEYSR

SEQ ID NO: 19 - protein, 16 aa, Homo sapiens
IAPQLSTEELVSLGEK

SEQ ID NO: 20 - protein, 14 aa, Homo sapiens
DIVLVAHSALGTQR

SEQ ID NO: 21 - protein, 19 aa, Homo sapiens
HIDSAYLYNNEEQVGLAIR

SEQ ID NO: 22 - protein, 12 aa, Homo sapiens
ADDGRPFPQVIK

SEQ ID NO: 23 - protein, 14 aa, Homo sapiens
GILAADESTGSIAK

SEQ ID NO: 24 - protein, 11 aa, Homo sapiens
EATDVIIIHSK

SEQ ID NO: 25 - protein, 14 aa, Homo sapiens
FSTEYELQQLEQFK

SEQ ID NO: 26 - protein, 9 aa, Homo sapiens
SIQLPTTVR

SEQ ID NO: 27 - protein, 16 aa, Homo sapiens
LLLTSAPSLATSPAFR

SEQ ID NO: 28 - protein, 13 aa, Homo sapiens
IVTATVNNSVLQK

SEQ ID NO: 29 - protein, 11 aa, Homo sapiens
QILDQTSEINK

SEQ ID NO: 30 - protein, 9 aa, Homo sapiens
AKPALEDLR

SEQ ID NO: 31 - protein, 11 aa, Homo sapiens
ATEHLSTLSEK

SEQ ID NO: 32 - protein, 13 aa, Homo sapiens
DYVSQFEGSALGK

SEQ ID NO: 33 - protein, 16 aa, Homo sapiens
EQLGPVTQEFWDNLEK

SEQ ID NO: 34 - protein, 11 aa, Homo sapiens
QGLLPVLESFK

SEQ ID NO: 35 - protein, 11 aa, Homo sapiens
THLAPYSDELR

SEQ ID NO: 36 - protein, 10 aa, Homo sapiens
VQPYLDDFQK

SEQ ID NO: 37 - protein, 12 aa, Homo sapiens
VSFLSALEEYTK

SEQ ID NO: 38 - protein, 13 aa, Homo sapiens
LGEVNTYAGDLQK

SEQ ID NO: 39 - protein, 14 aa, Homo sapiens
SELTQQLNALFQDK

SEQ ID NO: 40 - protein, 12 aa, Homo sapiens
SLAPYAQDTQEK

SEQ ID NO: 41 - protein, 16 aa, Homo sapiens
ELEGWEPDDDPIEEHK

SEQ ID NO: 42 - protein, 12 aa, Homo sapiens
QFEELTLGEFLK

SEQ ID NO: 43 - protein, 11 aa, Homo sapiens
EDVYVVGTVLR

SEQ ID NO: 44 - protein, 9 aa, Homo sapiens
GYILVGQAK

SEQ ID NO: 45 - protein, 12 aa, Homo sapiens
LSLEIEQLELQR

SEQ ID NO: 46 - protein, 9 aa, Homo sapiens
GLQTSQDAR

SEQ ID NO: 47 - protein, 8 aa, Homo sapiens
QIDNPDYK

SEQ ID NO: 48 - protein, 8 aa, Homo sapiens
VHVIFNYK

SEQ ID NO: 49 - protein, 10 aa, Homo sapiens
EQWPQCPTIK

SEQ ID NO: 50 - protein, 8 aa, Homo sapiens
LPASFDAR

SEQ ID NO: 51 - protein, 18 aa, Homo sapiens
NGPVEGAFSVYSDFLLYK

SEQ ID NO: 52 - protein, 18 aa, Homo sapiens
SGVYQHVTGEMMGGHAIR

SEQ ID NO: 53 - protein, 7 aa, Homo sapiens
TDQYWEK

SEQ ID NO: 54 - protein, 17 aa, Homo sapiens
GQDHCGIESEVVAGIPR

SEQ ID NO: 55 - protein, 20 aa, Homo sapiens
DQGSCGSCWAFGAVEAISDR

SEQ ID NO: 56 - protein, 14 aa, Homo sapiens
HYGYNSYSVSNSEK

SEQ ID NO: 57 - protein, 15 aa, Homo sapiens
GLVSGGLYESHVGCR

SEQ ID NO: 58 - protein, 22 aa, Homo sapiens
HYGYNSYSVSNSEKDIMAEIYK

SEQ ID NO: 59 - protein, 14 aa, Homo sapiens
ICEPGYSPTYKQDK

SEQ ID NO: 60 - protein, 25 aa, Homo sapiens
QDKHYGYNSYSVSNSEKDIMAEIYK

SEQ ID NO: 61 - protein, 11 aa, Homo sapiens
ICEPGYSPTYK

SEQ ID NO: 62 - protein, 17 aa, Homo sapiens
QDKHYGYNSYSVSNSEK

SEQ ID NO: 63 - protein, 8 aa, Homo sapiens
DIMAEIYK

SEQ ID NO: 64 - protein, 9 aa, Homo sapiens
AASQPGELK

SEQ ID NO: 65 - protein, 12 aa, Homo sapiens
NSLISYLEQIHR

SEQ ID NO: 66 - protein, 10 aa, Homo sapiens
SNAQGIDLNR

SEQ ID NO: 67 - protein, 9 aa, Homo sapiens
FAGVFHVEK

SEQ ID NO: 68 - protein, 12 aa, Homo sapiens
YGFIEGHVVIPR

SEQ ID NO: 69 - protein, 20 aa, Homo sapiens
AEEEHLGILGPQLHADVGDK

SEQ ID NO: 70 - protein, 12 aa, Homo sapiens
ALYLQYTDETFR

SEQ ID NO: 71 - protein, 13 aa, Homo sapiens
GAYPLSIEPIGVR

SEQ ID NO: 72 - protein, 16 aa, Homo sapiens
NNEGTYYSPNYNPQSR

SEQ ID NO: 73 - protein, 12 aa, Homo sapiens
ASSIIDELFQDR

SEQ ID NO: 74 - protein, 11 aa, Homo sapiens
ELDESLQVAER

SEQ ID NO: 75 - protein, 9 aa, Homo sapiens
IDSLLENDR

SEQ ID NO: 76 - protein, 17 aa, Homo sapiens
LFDSDPITVTVPVEVSR

SEQ ID NO: 77 - protein, 12 aa, Homo sapiens
GEPGNIGFPGPK

SEQ ID NO: 78 - protein, 15 aa, Homo sapiens
GIPGPVGAAGATGAR

SEQ ID NO: 79 - protein, 10 aa, Homo sapiens
IHWESASLLR

SEQ ID NO: 80 - protein, 16 aa, Homo sapiens
SNLDEDIIAEENIVSR

SEQ ID NO: 81 - protein, 12 aa, Homo sapiens
TIYTPGSTVLYR

SEQ ID NO: 82 - protein, 11 aa, Homo sapiens
LSIIATDHTYR

SEQ ID NO: 83 - protein, 9 aa, Homo sapiens
ADGVPVYLK

SEQ ID NO: 84 - protein, 9 aa, Homo sapiens
GLPDQMLYR

SEQ ID NO: 85 - protein, 13 aa, Homo sapiens
LTSDSTVYDYAGK

SEQ ID NO: 86 - protein, 16 aa, Homo sapiens
DFVEILDGGHEDAPLR

SEQ ID NO: 87 - protein, 17 aa, Homo sapiens
EQLANPIVSSGNSLFLR

SEQ ID NO: 88 - protein, 13 aa, Homo sapiens
FVTDGSVTASGFR

SEQ ID NO: 89 - protein, 11 aa, Homo sapiens
SDNSPTHVGFK

SEQ ID NO: 90 - protein, 20 aa, Homo sapiens
AAQAAVASYNMGSNSIYYFR

SEQ ID NO: 91 - protein, 10 aa, Homo sapiens
AQSQLVAGIK

SEQ ID NO: 92 - protein, 6 aa, Homo sapiens
ARPQER

SEQ ID NO: 93 - protein, 18 aa, Homo sapiens
CDFEVLVVPWQNSSQLLK

SEQ ID NO: 94 - protein, 11 aa, Homo sapiens
DLSPDDPQVQK

SEQ ID NO: 95 - protein, 6 aa, Homo sapiens
DTHIIK

SEQ ID NO: 96 - protein, 20 aa, Homo sapiens
LRCDFEVLVVPWQNSSQLLK

SEQ ID NO: 97 - protein, 21 aa, Homo sapiens
SNLPLALGLALVAFCLLALPR

SEQ ID NO: 98 - protein, 23 aa, Homo sapiens
TRVTGDHVDLTTCPLAAGAQQEK

SEQ ID NO: 99 - protein, 21 aa, Homo sapiens
VTGDHVDLTTCPLAAGAQQEK

SEQ ID NO: 100 - protein, 13 aa, Homo sapiens
YFLTMEMGSTDCR

SEQ ID NO: 101 - protein, 14 aa, Homo sapiens
YFLTMEMGSTDCRK

SEQ ID NO: 102 - protein, 14 aa, Homo sapiens
LGTFEVEDQIEAAR

SEQ ID NO: 103 - protein, 10 aa, Homo sapiens
VLEDNSALDK

SEQ ID NO: 104 - protein, 11 aa, Homo sapiens
WEYYDSVYTER

SEQ ID NO: 105 - protein, 11 aa, Homo sapiens
IESSSLQGLGR

SEQ ID NO: 106 - protein, 8 aa, Homo sapiens
IYWVDLER

SEQ ID NO: 107 - protein, 8 aa, Homo sapiens
LFWIQYNR

SEQ ID NO: 108 - protein, 11 aa, Homo sapiens
NQVTPLDILSK

SEQ ID NO: 109 - protein, 8 aa, Homo sapiens
LAINLLAK

SEQ ID NO: 110 - protein, 20 aa, Homo sapiens
LLDIESQEELEDFPLPTVQR

SEQ ID NO: 111 - protein, 18 aa, Homo sapiens
SQPVSQPLTYESGPDEVR

SEQ ID NO: 112 - protein, 9 aa, Homo sapiens
QDGSVDFFR

SEQ ID NO: 113 - protein, 9 aa, Homo sapiens
YGIDWASGR

SEQ ID NO: 114 - protein, 15 aa, Homo sapiens
DNENVVNEYSSELEK

SEQ ID NO: 115 - protein, 18 aa, Homo sapiens
HQLYIDETVNSNIPTNLR

SEQ ID NO: 116 - protein, 8 aa, Homo sapiens
IRPFFPQQ

SEQ ID NO: 117 - protein, 15 aa, Homo sapiens
IHLISTQSAIPYALR

SEQ ID NO: 118 - protein, 11 aa, Homo sapiens
QSGLYFIKPLK

SEQ ID NO: 119 - protein, 13 aa, Homo sapiens
YEASILTHDSSIR

SEQ ID NO: 120 - protein, 12 aa, Homo sapiens
AALPEGLPEASR

SEQ ID NO: 121 - protein, 9 aa, Homo sapiens
AANMHAQIK

SEQ ID NO: 122 - protein, 19 aa, Homo sapiens
ANQSWEDSNTDLVPAPAVR

SEQ ID NO: 123 - protein, 16 aa, Homo sapiens
ASLEDLGWADWVLSPR

SEQ ID NO: 124 - protein, 16 aa, Homo sapiens
EVQVTMCIGACPSQFR

SEQ ID NO: 125 - protein, 7 aa, Homo sapiens
ILTPEVR

SEQ ID NO: 126 - protein, 10 aa, Homo sapiens
LGSGGHLHLR

SEQ ID NO: 127 - protein, 24 aa, Homo sapiens
LKPDTVPAPCCVPASYNPMVLIQK

SEQ ID NO: 128 - protein, 7 aa, Homo sapiens
LSPTASR

SEQ ID NO: 129 - protein, 11 aa, Homo sapiens
NGDHCPLGPGR

SEQ ID NO: 130 - protein, 15 aa, Homo sapiens
QLSLARPQAPALHLR

SEQ ID NO: 131 - protein, 9 aa, Homo sapiens
SWDVTRPLR

SEQ ID NO: 132 - protein, 16 aa, Homo sapiens
TDTGVSLQTYDDLLAK

SEQ ID NO: 133 - protein, 21 aa, Homo sapiens
TDTGVSLQTYDDLLAKDCHCI

SEQ ID NO: 134 - protein, 7 aa, Homo sapiens
YEDLLTR

SEQ ID NO: 135 - protein, 13 aa, Homo sapiens
AGALNSNDAFVLK

SEQ ID NO: 136 - protein, 17 aa, Homo sapiens
QTQVSVLPEGGETPLFK

SEQ ID NO: 137 - protein, 9 aa, Homo sapiens
YIETDPANR

SEQ ID NO: 138 - protein, 12 aa, Homo sapiens
FFNVLTTNTDGK

SEQ ID NO: 139 - protein, 14 aa, Homo sapiens
TAFYLAEFFVNEAR

SEQ ID NO: 140 - protein, 12 aa, Homo sapiens
YPVYGVQWHPEK

SEQ ID NO: 141 - protein, 9 aa, Homo sapiens
ASWMPMFQR

SEQ ID NO: 142 - protein, 7 aa, Homo sapiens
CGMCCKT

SEQ ID NO: 143 - protein, 16 aa, Homo sapiens
DTHFPICIFCCGCCHR

SEQ ID NO: 144 - protein, 9 aa, Homo sapiens
SKCGMCCKT

SEQ ID NO: 145 - protein, 8 aa, Homo sapiens
LPGGLEPK

SEQ ID NO: 146 - protein, 14 aa, Homo sapiens
HEVTGWVLVSPLSK

SEQ ID NO: 147 - protein, 13 aa, Homo sapiens
ITVVDALHEIPVK

SEQ ID NO: 148 - protein, 8 aa, Homo sapiens
TELLPGDR

SEQ ID NO: 149 - protein, 15 aa, Homo sapiens
DVSTPPTVLPDNFPR

SEQ ID NO: 150 - protein, 14 aa, Homo sapiens
FNWYVDGVEVHNAK

SEQ ID NO: 151 - protein, 12 aa, Homo sapiens
GPSVFPLAPSSK

SEQ ID NO: 152 - protein, 17 aa, Homo sapiens
TTPPVLDSDGSFFLYSK

SEQ ID NO: 153 - protein, 11 aa, Homo sapiens
AVVEVDESGTR

SEQ ID NO: 154 - protein, 10 aa, Homo sapiens
EDQYHYLLDR

SEQ ID NO: 155 - protein, 15 aa, Homo sapiens
VEDLHVGATVAPSSR

SEQ ID NO: 156 - protein, 11 aa, Homo sapiens
FYNQVSTPLLR

SEQ ID NO: 157 - protein, 15 aa, Homo sapiens
IQPSGGTNINEALLR

SEQ ID NO: 158 - protein, 10 aa, Homo sapiens
TEVNVLPGAK

SEQ ID NO: 159 - protein, 9 aa, Homo sapiens
FAHTVVTSR

SEQ ID NO: 160 - protein, 12 aa, Homo sapiens
GPDVLTATVSGK

SEQ ID NO: 161 - protein, 9 aa, Homo sapiens
LGVYELLLK

SEQ ID NO: 162 - protein, 16 aa, Homo sapiens
SPEQQETVLDGNLIIR

SEQ ID NO: 163 - protein, 13 aa, Homo sapiens
AALEDTLAETEAR

SEQ ID NO: 164 - protein, 10 aa, Homo sapiens
ILGATIENSR

SEQ ID NO: 165 - protein, 17 aa, Homo sapiens
SLLEGQEDHYNNLSASK

SEQ ID NO: 166 - protein, 12 aa, Homo sapiens
LSEPAELTDAVK

SEQ ID NO: 167 - protein, 12 aa, Homo sapiens
LNAENNATFYFK

SEQ ID NO: 168 - protein, 11 aa, Homo sapiens
TVGSDTFYSFK

SEQ ID NO: 169 - protein, 8 aa, Homo sapiens
YFIDFVAR

SEQ ID NO: 170 - protein, 15 aa, Homo sapiens
YNSQNQSNNQFVLYR

SEQ ID NO: 171 - protein, 15 aa, Homo sapiens
AGQSPQLLIYTLSYR

SEQ ID NO: 172 - protein, 12 aa, Homo sapiens
LEIPYTFGQGTK

SEQ ID NO: 173 - protein, 11 aa, Homo sapiens
DAPSWDPVALK

SEQ ID NO: 174 - protein, 8 aa, Homo sapiens
LITEEANR

SEQ ID NO: 175 - protein, 14 aa, Homo sapiens
SGVLSVSSGAAAHR

SEQ ID NO: 176 - protein, 11 aa, Homo sapiens
ALQATVGNSYK

SEQ ID NO: 177 - protein, 16 aa, Homo sapiens
FFLQGIQLNTILPDAR

SEQ ID NO: 178 - protein, 10 aa, Homo sapiens
GHTLTLNFTR

SEQ ID NO: 179 - protein, 12 aa, Homo sapiens
GILTVDELLAIR

SEQ ID NO: 180 - protein, 9 aa, Homo sapiens
YLDFVFAVK

SEQ ID NO: 181 - protein, 15 aa, Homo sapiens
DLADELALVDVIEDK

SEQ ID NO: 182 - protein, 10 aa, Homo sapiens
SADTLWGIQK

SEQ ID NO: 183 - protein, 10 aa, Homo sapiens
VTLTSEEEAR

SEQ ID NO: 184 - protein, 14 aa, Homo sapiens
ELSEALGQIFDSQR

SEQ ID NO: 185 - protein, 9 aa, Homo sapiens
IDITLSSVK

SEQ ID NO: 186 - protein, 11 aa, Homo sapiens
LADGGATNQGR

SEQ ID NO: 187 - protein, 13 aa, Homo sapiens
SDLAVPSELALLK

SEQ ID NO: 188 - protein, 13 aa, Homo sapiens
YSSDYFQAPSDYR

SEQ ID NO: 189 - protein, 10 aa, Homo sapiens
ELAPLFEELR

SEQ ID NO: 190 - protein, 15 aa, Homo sapiens
LPSVEGLHAIVVSDR

SEQ ID NO: 191 - protein, 11 aa, Homo sapiens
GAYTQVIFLAR

SEQ ID NO: 192 - protein, 16 aa, Homo sapiens
GELFWDDGESLEVLER

SEQ ID NO: 193 - protein, 10 aa, Homo sapiens
WGYSSTAITR

SEQ ID NO: 194 - protein, 9 aa, Homo sapiens
DFADIPNLR

SEQ ID NO: 195 - protein, 11 aa, Homo sapiens
AAYEDFNVQLR

SEQ ID NO: 196 - protein, 14 aa, Homo sapiens
AVTLSLDGGDTAIR

SEQ ID NO: 197 - protein, 9 aa, Homo sapiens
DGNVFLVPK

SEQ ID NO: 198 - protein, 12 aa, Homo sapiens
EQFNEAQLALIR

SEQ ID NO: 199 - protein, 8 aa, Homo sapiens
DGVVSVNK

SEQ ID NO: 200 - protein, 12 aa, Homo sapiens
ESYNVQLQLPAR

SEQ ID NO: 201 - protein, 12 aa, Homo sapiens
HAQAQYAYPGAR

SEQ ID NO: 202 - protein, 17 aa, Homo sapiens
AIPVAQDLNAPSDWDSR

SEQ ID NO: 203 - protein, 19 aa, Homo sapiens
ANDESNEHSDVIDSQELSK

SEQ ID NO: 204 - protein, 16 aa, Homo sapiens
YPDAVATWLNPDPSQK

SEQ ID NO: 205 - protein, 10 aa, Homo sapiens
LGFLHSGTAK

SEQ ID NO: 206 - protein, 18 aa, Homo sapiens
LLEIDSVGSEDSLDTSLR

SEQ ID NO: 207 - protein, 8 aa, Homo sapiens
TVIYEIPR

SEQ ID NO: 208 - protein, 11 aa, Homo sapiens
IQAIELEDLLR

SEQ ID NO: 209 - protein, 14 aa, Homo sapiens
LLQVVYLHSNNITK

SEQ ID NO: 210 - protein, 18 aa, Homo sapiens
NHLVEIPPNLPSSLVELR

SEQ ID NO: 211 - protein, 18 aa, Homo sapiens
ASPATLLLVLCLQLGANK

SEQ ID NO: 212 - protein, 15 aa, Homo sapiens
ELGICPDDAAVIPIK

SEQ ID NO: 213 - protein, 18 aa, Homo sapiens
ELGICPDDAAVIPIKNNR

SEQ ID NO: 214 - protein, 8 aa, Homo sapiens
FYTIEILK

SEQ ID NO: 215 - protein, 10 aa, Homo sapiens
FYTIEILKVE

SEQ ID NO: 216 - protein, 7 aa, Homo sapiens
LLQLLFR

SEQ ID NO: 217 - protein, 6 aa, Homo sapiens
NFDIPK

SEQ ID NO: 218 - protein, 19 aa, Homo sapiens
SVRPNDEVTAVLAVQTELK

SEQ ID NO: 219 - protein, 25 aa, Homo sapiens
SVRPNDEVTAVLAVQTELKECMVVK

SEQ ID NO: 220 - protein, 10 aa, Homo sapiens
TFYWDFYTNR

SEQ ID NO: 221 - protein, 12 aa, Homo sapiens
TVQIAAVVDVIR

SEQ ID NO: 222 - protein, 16 aa, Homo sapiens
TYLISSIPLQGAFNYK

SEQ ID NO: 223 - protein, 11 aa, Homo sapiens
YTACLCDDNPK

SEQ ID NO: 224 - protein, 12 aa, Homo sapiens
AGALQLLLVGDK

SEQ ID NO: 225 - protein, 20 aa, Homo sapiens
ATYFGSIVLLSPAVIDSPLK

SEQ ID NO: 226 - protein, 12 aa, Homo sapiens
EGHFYYNISEVK

SEQ ID NO: 227 - protein, 15 aa, Homo sapiens
ELSELSLLSLYGIHK

SEQ ID NO: 228 - protein, 10 aa, Homo sapiens
FQELESETLK

SEQ ID NO: 229 - protein, 12 aa, Homo sapiens
SPIDTFPTDPIK

SEQ ID NO: 230 - protein, 12 aa, Homo sapiens
ADLHAVQGWAAR

SEQ ID NO: 231 - protein, 11 aa, Homo sapiens
MLLQATDDVLR

SEQ ID NO: 232 - protein, 16 aa, Homo sapiens
SWLPAGCETAILFPMR

SEQ ID NO: 233 - protein, 14 aa, Homo sapiens
AEQWNVNYVETSAK

SEQ ID NO: 234 - protein, 13 aa, Homo sapiens
EDENVPFLLVGNK

SEQ ID NO: 235 - protein, 9 aa, Homo sapiens
GQNSLALHK

SEQ ID NO: 236 - protein, 9 aa, Homo sapiens
SFEDIHHYR

SEQ ID NO: 237 - protein, 10 aa, Homo sapiens
VEDAFYTLVR

SEQ ID NO: 238 - protein, 9 aa, Homo sapiens
SFADINLYR

SEQ ID NO: 239 - protein, 11 aa, Homo sapiens
DPNGLPPEAQK

SEQ ID NO: 240 - protein, 14 aa, Homo sapiens
DPNGLPPEAQKIVR

SEQ ID NO: 241 - protein, 10 aa, Homo sapiens
FSGTWYAMAK

SEQ ID NO: 242 - protein, 22 aa, Homo sapiens
GNDDHWIVDTDYDTYAVQYSCR

SEQ ID NO: 243 - protein, 29 aa, Homo sapiens
KDPEGLFLQDNIVAEFSVDETGQMSATAK

SEQ ID NO: 244 - protein, 11 aa, Homo sapiens
LIVHNGYCDGR

SEQ ID NO: 245 - protein, 14 aa, Homo sapiens
LIVHNGYCDGRSER

SEQ ID NO: 246 - protein, 18 aa, Homo sapiens
LLNLDGTCADSYSFVFSR

SEQ ID NO: 247 - protein, 23 aa, Homo sapiens
LLNNWDVCADMVGTFTDTEDPAK

SEQ ID NO: 248 - protein, 25 aa, Homo sapiens
LLNNWDVCADMVGTFTDTEDPAKFK

SEQ ID NO: 249 - protein, 12 aa, Homo sapiens
MKYWGVASFLQK

SEQ ID NO: 250 - protein, 8 aa, Homo sapiens
QEELCLAR

SEQ ID NO: 251 - protein, 10 aa, Homo sapiens
QRQEELCLAR

SEQ ID NO: 252 - protein, 9 aa, Homo sapiens
VKENFDKAR

SEQ ID NO: 253 - protein, 15 aa, Homo sapiens
WVWALLLLAALGSGR

SEQ ID NO: 254 - protein, 10 aa, Homo sapiens
YWGVASFLQK

SEQ ID NO: 255 - protein, 11 aa, Homo sapiens
IQEVAGSLIFR

SEQ ID NO: 256 - protein, 10 aa, Homo sapiens
DKDAVDKLLK

SEQ ID NO: 257 - protein, 28 aa, Homo sapiens
DLDANGDAQVDFSEFIVFVAAITSACHK

SEQ ID NO: 258 - protein, 10 aa, Homo sapiens
ELPGFLQSGK

SEQ ID NO: 259 - protein, 17 aa, Homo sapiens
ELPGFLQSGKDKDAVDK

SEQ ID NO: 260 - protein, 17 aa, Homo sapiens
MTELETAMGMIIDVFSR

SEQ ID NO: 261 - protein, 16 aa, Homo sapiens
TELETAMGMIIDVFSR

SEQ ID NO: 262 - protein, 13 aa, Homo sapiens
YSGSEGSTQTLTK

SEQ ID NO: 263 - protein, 17 aa, Homo sapiens
YSGSEGSTQTLTKGELK

SEQ ID NO: 264 - protein, 7 aa, Homo sapiens
LMEDLDR

SEQ ID NO: 265 - protein, 8 aa, Homo sapiens
LQDAEIAR

SEQ ID NO: 266 - protein, 9 aa, Homo sapiens
AADLLLHSK

SEQ ID NO: 267 - protein, 13 aa, Homo sapiens
ITTVSLSAPDALK

SEQ ID NO: 268 - protein, 12 aa, Homo sapiens
TNVYISSSAGAR

SEQ ID NO: 269 - protein, 15 aa, Homo sapiens
ELQELVQYPVEHPDK

SEQ ID NO: 270 - protein, 10 aa, Homo sapiens
GDDLSTAILK

SEQ ID NO: 271 - protein, 20 aa, Homo sapiens
LIVDEAINEDNSVVSLSQPK

SEQ ID NO: 272 - protein, 17 aa, Homo sapiens
GQGCPSTHVLLTHTISR

SEQ ID NO: 273 - protein, 8 aa, Homo sapiens
VNLLSAIK

SEQ ID NO: 274 - protein, 10 aa, Homo sapiens
DGAGDVAFVK

SEQ ID NO: 275 - protein, 11 aa, Homo sapiens
EGYYGYTGAFR

SEQ ID NO: 276 - protein, 11 aa, Homo sapiens
SASDLTWDNLK

SEQ ID NO: 277 - protein, 15 aa, Homo sapiens
GGVNDNFQGVLQNVR

SEQ ID NO: 278 - protein, 11 aa, Homo sapiens
TIVTTLQDSIR

SEQ ID NO: 279 - protein, 16 aa, Homo sapiens
DSTIQVVENGESSQGR

SEQ ID NO: 280 - protein, 10 aa, Homo sapiens
DWVSVVTPAR

SEQ ID NO: 281 - protein, 13 aa, Homo sapiens
EDFTSLSLVLYSR

SEQ ID NO: 282 - protein, 10 aa, Homo sapiens
THLPEVFLSK

SEQ ID NO: 283 - protein, 7 aa, Homo sapiens
YTFELSR

SEQ ID NO: 284 - protein, 16 aa, Homo sapiens
EIPAWVPFDPAAQITK

SEQ ID NO: 285 - protein, 10 aa, Homo sapiens
WEAEPVYVQR

SEQ ID NO: 286 - protein, 12 aa, Homo sapiens
YSLTYIYTGLSK

SEQ ID NO: 287 - protein, 12 aa, Homo sapiens
TLMFGSYLDDEK

SEQ ID NO: 288 - protein, 17 aa, Homo sapiens
EQLGEFYEALDCLCIPR

SEQ ID NO: 289 - protein, 15 aa, Homo sapiens
QNQCFYNSSYLNVQR

SEQ ID NO: 290 - protein, 8 aa, Homo sapiens
LLELTGPK

SEQ ID NO: 291 - protein, 16 aa, Homo sapiens
NGVAQEPVHLDSPAIK

SEQ ID NO: 292 - protein, 12 aa, Homo sapiens
SGLSTGWTQLSK

SEQ ID NO: 293 - protein, 16 aa, Homo sapiens
ENQLEVLEVSWLHGLK

SEQ ID NO: 294 - protein, 7 aa, Homo sapiens
GPLQLER

SEQ ID NO: 295 - protein, 10 aa, Homo sapiens
GHFSISIPVK

SEQ ID NO: 296 - protein, 12 aa, Homo sapiens
HYDGSYSTFGER

SEQ ID NO: 297 - protein, 9 aa, Homo sapiens
AIPVTQYLK

SEQ ID NO: 298 - protein, 9 aa, Homo sapiens
LPNNVLQEK

SEQ ID NO: 299 - protein, 7 aa, Homo sapiens
VLDGLNR

SEQ ID NO: 300 - protein, 17 aa, Homo sapiens
VIFDTVDLSATWEVMEK

SEQ ID NO: 301 - protein, 10 aa, Homo sapiens
DHSAIPVINR

SEQ ID NO: 302 - protein, 7 aa, Homo sapiens
ELWILNR

SEQ ID NO: 303 - protein, 15 aa, Homo sapiens
AQIINDAFNLASAHK

SEQ ID NO: 304 - protein, 7 aa, Homo sapiens
IQTQLQR

SEQ ID NO: 305 - protein, 16 aa, Homo sapiens
LLGPGPAADFSVSVER

SEQ ID NO: 306 - protein, 11 aa, Homo sapiens
FLLGSWLEQAR

SEQ ID NO: 307 - protein, 8 aa, Homo sapiens
YDLLDLTR

SEQ ID NO: 308 - protein, 8 aa, Homo sapiens
SDVFEAWR

SEQ ID NO: 309 - protein, 9 aa, Homo sapiens
VNSFFSTFK

SEQ ID NO: 310 - protein, 10 aa, Homo sapiens
ALVQQMEQLR

SEQ ID NO: 311 - protein, 9 aa, Homo sapiens
LGPLVEQGR

SEQ ID NO: 312 - protein, 15 aa, Homo sapiens
SELEEQLTPVAEETR

SEQ ID NO: 313 - protein, 10 aa, Homo sapiens
QQTEWQSGQR

SEQ ID NO: 314 - protein, 7 aa, Homo sapiens
WELALGR

SEQ ID NO: 315 - protein, 9 aa, Homo sapiens
LEEQAQQIR

SEQ ID NO: 316 - protein, 9 aa, Homo sapiens
LAVYQAGAR

SEQ ID NO: 317 - protein, 9 aa, Homo sapiens
HDLGHFMLR

SEQ ID NO: 318 - protein, 10 aa, Homo sapiens
LQAVTDDHIR

SEQ ID NO: 319 - protein, 15 aa, Homo sapiens
TVAGQDAVIVLLGTR

SEQ ID NO: 320 - protein, 14 aa, Homo sapiens
NDLSPTTVMSEGAR

SEQ ID NO: 321 - protein, 15 aa, Homo sapiens
VVACTSAFLLWDPTK

SEQ ID NO: 322 - protein, 15 aa, Homo sapiens
GVGWSHPLPQCEIVK

SEQ ID NO: 323 - protein, 10 aa, Homo sapiens
LNNGEITQHR

SEQ ID NO: 324 - protein, 9 aa, Homo sapiens
EEIIYECDK

SEQ ID NO: 325 - protein, 12 aa, Homo sapiens
GSSVIHCDADSK

SEQ ID NO: 326 - protein, 18 aa, Homo sapiens
DTANWLEINPDTGAISTR

SEQ ID NO: 327 - protein, 16 aa, Homo sapiens
GQVPENEANVVITTLK

SEQ ID NO: 328 - protein, 14 aa, Homo sapiens
NTGVISVVTTGLDR

SEQ ID NO: 329 - protein, 10 aa, Homo sapiens
VGTDGVITVK

SEQ ID NO: 330 - protein, 7 aa, Homo sapiens
VTEPLDR

SEQ ID NO: 331 - protein, 12 aa, Homo sapiens
EQFLDGDGWTSR

SEQ ID NO: 332 - protein, 11 aa, Homo sapiens
GQTLVVQFTVK

SEQ ID NO: 333 - protein, 14 aa, Homo sapiens
FYALSASFEPFSNK

SEQ ID NO: 334 - protein, 13 aa, Homo sapiens
HEQNIDCGGGYVK

SEQ ID NO: 335 - protein, 18 aa, Homo sapiens
YSQAVPAVTEGPIPEVLK

SEQ ID NO: 336 - protein, 13 aa, Homo sapiens
LVDQNIFSFYLSR

SEQ ID NO: 337 - protein, 10 aa, Homo sapiens
VSTLPAITLK

SEQ ID NO: 338 - protein, 8 aa, Homo sapiens
QVFGEATK

SEQ ID NO: 339 - protein, 7 aa, Homo sapiens
YYTVFDR

SEQ ID NO: 340 - protein, 10 aa, Homo sapiens
QPGITFIAAK

SEQ ID NO: 341 - protein, 9 aa, Homo sapiens
LSPEDYTLK

SEQ ID NO: 342 - protein, 9 aa, Homo sapiens
QVMNGFQNR

SEQ ID NO: 343 - protein, 23 aa, Homo sapiens
AVATVGPISVAIDAGHESFLFYK

SEQ ID NO: 344 - protein, 12 aa, Homo sapiens
VFQEPLFYEAPR

SEQ ID NO: 345 - protein, 14 aa, Homo sapiens
YSVANDTGFVDIPK

SEQ ID NO: 346 - protein, 14 aa, Homo sapiens
NSWGEEWGMGGYVK

SEQ ID NO: 347 - protein, 10 aa, Homo sapiens
MIELHNQEYR

SEQ ID NO: 348 - protein, 11 aa, Homo sapiens
LYGMNEEGWRR

SEQ ID NO: 349 - protein, 14 aa, Homo sapiens
NHCGIASAASYPTV

SEQ ID NO: 350 - protein, 8 aa, Homo sapiens
AGLQVYNK

SEQ ID NO: 351 - protein, 12 aa, Homo sapiens
FEHCNFNDVTTR

SEQ ID NO: 352 - protein, 16 aa, Homo sapiens
TAVNCSSDFDACLITK

SEQ ID NO: 353 - protein, 10 aa, Homo sapiens
ENELTYYCCK

SEQ ID NO: 354 - protein, 18 aa, Homo sapiens
TVLLLVTPFLAAAWSLHP

SEQ ID NO: 355 - protein, 18 aa, Homo sapiens
GANGAPGIAGAPGFPGAR

SEQ ID NO: 356 - protein, 10 aa, Homo sapiens
SLSQQIENIR

SEQ ID NO: 357 - protein, 9 aa, Homo sapiens
GFSGLDGAK

SEQ ID NO: 358 - protein, 13 aa, Homo sapiens
ALLLQGSNEIEIR

SEQ ID NO: 359 - protein, 9 aa, Homo sapiens
GSEGPQGVR

SEQ ID NO: 360 - protein, 9 aa, Homo sapiens
GEAGPQGPR

SEQ ID NO: 361 - protein, 9 aa, Homo sapiens
GVVGPQGAR

SEQ ID NO: 362 - protein, 13 aa, Homo sapiens
VYCDFSTGETCIR

SEQ ID NO: 363 - protein, 10 aa, Homo sapiens
EMATQLAFMR

SEQ ID NO: 364 - protein, 16 aa, Homo sapiens
SLNNQIETLLTPEGSR

SEQ ID NO: 365 - protein, 9 aa, Homo sapiens
TGLQEVEVK

SEQ ID NO: 366 - protein, 13 aa, Homo sapiens
SSLSVPYVIVPLK

SEQ ID NO: 367 - protein, 14 aa, Homo sapiens
VFSVAITPDHLEPR

SEQ ID NO: 368 - protein, 9 aa, Homo sapiens
IALVITDGR

SEQ ID NO: 369 - protein, 13 aa, Homo sapiens
ENYAELLEDAFLK

SEQ ID NO: 370 - protein, 9 aa, Homo sapiens
VPSYQALLR

SEQ ID NO: 371 - protein, 24 aa, Homo sapiens
TTMALTVGGTIYCLIALYMASQPK

SEQ ID NO: 372 - protein, 9 aa, Homo sapiens
IEPNLPSYR

SEQ ID NO: 373 - protein, 10 aa, Homo sapiens
WISDHEYLYK

SEQ ID NO: 374 - protein, 16 aa, Homo sapiens
TQNDVDIADVAYYFEK

SEQ ID NO: 375 - protein, 11 aa, Homo sapiens
LAVNCFVNNNR

SEQ ID NO: 376 - protein, 9 aa, Homo sapiens
TYWIIIELK

SEQ ID NO: 377 - protein, 8 aa, Homo sapiens
GESLFHSK

SEQ ID NO: 378 - protein, 23 aa, Homo sapiens
FITSILYENNVITIDLVQNSSQK

SEQ ID NO: 379 - protein, 13 aa, Homo sapiens
VGPQVPLSEPGFR

SEQ ID NO: 380 - protein, 20 aa, Homo sapiens
NTEISFILGQEFDEVTADDR

SEQ ID NO: 381 - protein, 9 aa, Homo sapiens
EVGVGFATR

SEQ ID NO: 382 - protein, 15 aa, Homo sapiens
STITLDGGVLVHVQK

SEQ ID NO: 383 - protein, 21 aa, Homo sapiens
VAGMAKPNMIISVNGDVITIK

SEQ ID NO: 384 - protein, 11 aa, Homo sapiens
GEPGDPVNLLR

SEQ ID NO: 385 - protein, 13 aa, Homo sapiens
YYWGGQYTWDMAK

SEQ ID NO: 386 - protein, 15 aa, Homo sapiens
NYCGLPGEYWLGNDK

SEQ ID NO: 387 - protein, 15 aa, Homo sapiens
EVQGFESATFLGYFK

SEQ ID NO: 388 - protein, 8 aa, Homo sapiens
TGAQELLR

SEQ ID NO: 389 - protein, 8 aa, Homo sapiens
YLESAGAR

SEQ ID NO: 390 - protein, 9 aa, Homo sapiens
YYIAASYVK

SEQ ID NO: 391 - protein, 13 aa, Homo sapiens
NLDGISHAPNAVK

SEQ ID NO: 392 - protein, 11 aa, Homo sapiens
IEFISTMEGYK

SEQ ID NO: 393 - protein, 9 aa, Homo sapiens
MFLSFPTTK

SEQ ID NO: 394 - protein, 16 aa, Homo sapiens
TYFPHFDLSHGSAQVK

SEQ ID NO: 395 - protein, 15 aa, Homo sapiens
VGAHAGEYGAEALER

SEQ ID NO: 396 - protein, 12 aa, Homo sapiens
FLASVSTVLTSK

SEQ ID NO: 397 - protein, 19 aa, Homo sapiens
FFESFGDLSTPDAVMGNPK

SEQ ID NO: 398 - protein, 9 aa, Homo sapiens
SAVTALWGK

SEQ ID NO: 399 - protein, 13 aa, Homo sapiens
VNVDEVGGEALGR

SEQ ID NO: 400 - protein, 12 aa, Homo sapiens
EFTPPVQAAYQK

SEQ ID NO: 401 - protein, 13 aa, Homo sapiens
GTFATLSELHCDK

SEQ ID NO: 402 - protein, 9 aa, Homo sapiens
VGYVSGWGR

SEQ ID NO: 403 - protein, 10 aa, Homo sapiens
VTSIQDWVQK

SEQ ID NO: 404 - protein, 16 aa, Homo sapiens
VVLHPNYSQVDIGLIK

SEQ ID NO: 405 - protein, 7 aa, Homo sapiens
DYAEVGR

SEQ ID NO: 406 - protein, 10 aa, Homo sapiens
HYEGSTVPEK

SEQ ID NO: 407 - protein, 15 aa, Homo sapiens
THEDLYIIPIPNCDR

SEQ ID NO: 408 - protein, 7 aa, Homo sapiens
LAASQSR

SEQ ID NO: 409 - protein, 17 aa, Homo sapiens
EDARPVPQGSCQSELHR

SEQ ID NO: 410 - protein, 7 aa, Homo sapiens
NGNFHPK

SEQ ID NO: 411 - protein, 10 aa, Homo sapiens
APAVAEENPK

SEQ ID NO: 412 - protein, 15 aa, Homo sapiens
HLDSVLQQLQTEVYR

SEQ ID NO: 413 - protein, 13 aa, Homo sapiens
GAQTLYVPNCDHR

SEQ ID NO: 414 - protein, 23 aa, Homo sapiens
LLPPLLLLLALLLAASPGGALAR

SEQ ID NO: 415 - protein, 7 aa, Homo sapiens
DDEAPLR

SEQ ID NO: 416 - protein, 16 aa, Homo sapiens
ESKPQAGTARPQDVNR

SEQ ID NO: 417 - protein, 12 aa, Homo sapiens
LGELILTSESSR

SEQ ID NO: 418 - protein, 10 aa, Homo sapiens
QADSDIPLDR

SEQ ID NO: 419 - protein, 14 aa, Homo sapiens
FHLATAEWIAEPVR

SEQ ID NO: 420 - protein, 13 aa, Homo sapiens
LYPESQGSDTAWR

SEQ ID NO: 421 - protein, 11 aa, Homo sapiens
SSGPGGQNVNK

SEQ ID NO: 422 - protein, 19 aa, Homo sapiens
TPEVTCVVVDVSHEDPEVK

SEQ ID NO: 423 - protein, 12 aa, Homo sapiens
EALAENNLNLPK

SEQ ID NO: 424 - protein, 8 aa, Homo sapiens
EFLQSSLR

SEQ ID NO: 425 - protein, 9 aa, Homo sapiens
FESSEEQAR

SEQ ID NO: 426 - protein, 18 aa, Homo sapiens
IITGLLEFEVYLEYLQNR

SEQ ID NO: 427 - protein, 18 aa, Homo sapiens
LQAQNQWLQDMTTHLILR

SEQ ID NO: 428 - protein, 19 aa, Homo sapiens
NLDAITTPDPTTNASLLTK

SEQ ID NO: 429 - protein, 8 aa, Homo sapiens
QPLTSSER

SEQ ID NO: 430 - protein, 10 aa, Homo sapiens
YILDGISALR

SEQ ID NO: 431 - protein, 16 aa, Homo sapiens
DGCFQSGFNEETCLVK

SEQ ID NO: 432 - protein, 8 aa, Homo sapiens
VLIQFLQK

SEQ ID NO: 433 - protein, 15 aa, Homo sapiens
LLGASELPIVTPALR

SEQ ID NO: 434 - protein, 9 aa, Homo sapiens
TGVVPQLVK

SEQ ID NO: 435 - protein, 18 aa, Homo sapiens
IILVILDAISNIFQAAEK

SEQ ID NO: 436 - protein, 8 aa, Homo sapiens
ASLSLIEK

SEQ ID NO: 437 - protein, 15 aa, Homo sapiens
NNQGTVNWSVDDIVK

SEQ ID NO: 438 - protein, 11 aa, Homo sapiens
FSIEGSYQLEK

SEQ ID NO: 439 - protein, 21 aa, Homo sapiens
VVGVPYQGNATALFILPSEGK

SEQ ID NO: 440 - protein, 13 aa, Homo sapiens
MQILEGLGLNLQK

SEQ ID NO: 441 - protein, 8 aa, Homo sapiens
VQSTITSR

SEQ ID NO: 442 - protein, 8 aa, Homo sapiens
NDLISATK

SEQ ID NO: 443 - protein, 7 aa, Homo sapiens
TILDDLR

SEQ ID NO: 444 - protein, 11 aa, Homo sapiens
VQFELHYQEVK

SEQ ID NO: 445 - protein, 9 aa, Homo sapiens
AFDSDGDGR

SEQ ID NO: 446 - protein, 7 aa, Homo sapiens
YSFLELR

SEQ ID NO: 447 - protein, 11 aa, Homo sapiens
FSQFLGDPVEK

SEQ ID NO: 448 - protein, 21 aa, Homo sapiens
LTYQEIWTSLGSAMPEPESLR

SEQ ID NO: 449 - protein, 17 aa, Homo sapiens
SAADLISLPTTVEGLQK

SEQ ID NO: 450 - protein, 13 aa, Homo sapiens
QISLLTSAVNHLK

SEQ ID NO: 451 - protein, 12 aa, Homo sapiens
ALEEANTELEVK

SEQ ID NO: 452 - protein, 12 aa, Homo sapiens
LSVEADINGLRR

SEQ ID NO: 453 - protein, 8 aa, Homo sapiens
TIEELQNK

SEQ ID NO: 454 - protein, 13 aa, Homo sapiens
ASLEGNLAETENR

SEQ ID NO: 455 - protein, 10 aa, Homo sapiens
TIVEEVQDGK

SEQ ID NO: 456 - protein, 8 aa, Homo sapiens
FGPGVAFR

SEQ ID NO: 457 - protein, 12 aa, Homo sapiens
ALEAANGELEVK

SEQ ID NO: 458 - protein, 21 aa, Homo sapiens
SSQSLLDSGDGNTYLNWYLQK

SEQ ID NO: 459 - protein, 14 aa, Homo sapiens
VQAEDVGVYYCMQR

SEQ ID NO: 460 - protein, 9 aa, Homo sapiens
TVESITDIR

SEQ ID NO: 461 - protein, 8 aa, Homo sapiens
AFSVNIFK

SEQ ID NO: 462 - protein, 14 aa, Homo sapiens
ENTSDPSLVIAFGR

SEQ ID NO: 463 - protein, 16 aa, Homo sapiens
NMTFDLPSDATVVLNR

SEQ ID NO: 464 - protein, 12 aa, Homo sapiens
VTSEGAGLQLQK

SEQ ID NO: 465 - protein, 17 aa, Homo sapiens
STGGILDVYIFLGPEPK

SEQ ID NO: 466 - protein, 9 aa, Homo sapiens
GTRPFVISR

SEQ ID NO: 467 - protein, 13 aa, Homo sapiens
YEVPLETPHVHSR

SEQ ID NO: 468 - protein, 15 aa, Homo sapiens
TDDIGTASGWGLTQR

SEQ ID NO: 469 - protein, 8 aa, Homo sapiens
ESAYLYAR

SEQ ID NO: 470 - protein, 10 aa, Homo sapiens
LEGNPIVLGK

SEQ ID NO: 471 - protein, 7 aa, Homo sapiens
LTLFNAK

SEQ ID NO: 472 - protein, 9 aa, Homo sapiens
HPNSFICLK

SEQ ID NO: 473 - protein, 9 aa, Homo sapiens
FQTFEGDLK

SEQ ID NO: 474 - protein, 15 aa, Homo sapiens
LGLGADVAQVTGALR

SEQ ID NO: 475 - protein, 16 aa, Homo sapiens
QLSLPETGELDSATLK

SEQ ID NO: 476 - protein, 12 aa, Homo sapiens
QSTLVLFPGDLR

SEQ ID NO: 477 - protein, 10 aa, Homo sapiens
SYSACTTDGR

SEQ ID NO: 478 - protein, 15 aa, Homo sapiens
DISSSLNSLADSNAR

SEQ ID NO: 479 - protein, 9 aa, Homo sapiens
LVEGESDNR

SEQ ID NO: 480 - protein, 10 aa, Homo sapiens
TLLADQGEIR

SEQ ID NO: 481 - protein, 11 aa, Homo sapiens
QFESLPATHIR

SEQ ID NO: 482 - protein, 18 aa, Homo sapiens
VGDYVYFENSSSNPYLVR

SEQ ID NO: 483 - protein, 16 aa, Homo sapiens
EFEEESKQPGVSEQQR

SEQ ID NO: 484 - protein, 11 aa, Homo sapiens
LTPLQFGNLQK

SEQ ID NO: 485 - protein, 13 aa, Homo sapiens
TGLLVEQSGDYIK

SEQ ID NO: 486 - protein, 16 aa, Homo sapiens
LFVESYELILQEGTFK

SEQ ID NO: 487 - protein, 14 aa, Homo sapiens
SVVGDALEFGNSWK

SEQ ID NO: 488 - protein, 12 aa, Homo sapiens
ELLNETEEEINK

SEQ ID NO: 489 - protein, 8 aa, Homo sapiens
LFLDYTIK

SEQ ID NO: 490 - protein, 9 aa, Homo sapiens
LQNIIDNQK

SEQ ID NO: 491 - protein, 9 aa, Homo sapiens
NELQQTINK

SEQ ID NO: 492 - protein, 12 aa, Homo sapiens
NSQLGIFSSSEK

SEQ ID NO: 493 - protein, 10 aa, Homo sapiens
QHGDVVSAIR

SEQ ID NO: 494 - protein, 14 aa, Homo sapiens
SVDPDSPAEASGLR

SEQ ID NO: 495 - protein, 13 aa, Homo sapiens
GPNGYGFHLHGEK

SEQ ID NO: 496 - protein, 10 aa, Homo sapiens
LVEPGSPAEK

SEQ ID NO: 497 - protein, 17 aa, Homo sapiens
EALAEAALESPRPALVR

SEQ ID NO: 498 - protein, 12 aa, Homo sapiens
IVEVNGVCMEGK

SEQ ID NO: 499 - protein, 8 aa, Homo sapiens
EEDTGRPR

SEQ ID NO: 500 - protein, 8 aa, Homo sapiens
SDHPAILR

SEQ ID NO: 501 - protein, 9 aa, Homo sapiens
GFSGIFEDR

SEQ ID NO: 502 - protein, 15 aa, Homo sapiens
LLGEVGTLQFAELHR

SEQ ID NO: 503 - protein, 11 aa, Homo sapiens
EVDSDAYYVYR

SEQ ID NO: 504 - protein, 17 aa, Homo sapiens
LVEPVTDFLLDMPYHIR

SEQ ID NO: 505 - protein, 15 aa, Homo sapiens
DLPETLNELHLDHNK

SEQ ID NO: 506 - protein, 14 aa, Homo sapiens
GLQHLYALVLVNNK

SEQ ID NO: 507 - protein, 10 aa, Homo sapiens
VVQCSDLGLK

SEQ ID NO: 508 - protein, 9 aa, Homo sapiens
VPSGLPDLK

SEQ ID NO: 509 - protein, 12 aa, Homo sapiens
HINPVAASLIQK

SEQ ID NO: 510 - protein, 13 aa, Homo sapiens
LGNLFLNEDLEVK

SEQ ID NO: 511 - protein, 15 aa, Homo sapiens
LILYNDGDSLQYIER

SEQ ID NO: 512 - protein, 13 aa, Homo sapiens
FSIAPSSLDPSNR

SEQ ID NO: 513 - protein, 9 aa, Homo sapiens
IGDFGLATK

SEQ ID NO: 514 - protein, 8 aa, Homo sapiens
AGANITPR

SEQ ID NO: 515 - protein, 11 aa, Homo sapiens
GLENPLPERPR

SEQ ID NO: 516 - protein, 10 aa, Homo sapiens
MHAAFGGTFK

SEQ ID NO: 517 - protein, 8 aa, Homo sapiens
DISLSDYK

SEQ ID NO: 518 - protein, 8 aa, Homo sapiens
ADEGISFR

SEQ ID NO: 519 - protein, 11 aa, Homo sapiens
ATAVMPDGQFK

SEQ ID NO: 520 - protein, 16 aa, Homo sapiens
QGGLGPMNIPLVSDPK

SEQ ID NO: 521 - protein, 10 aa, Homo sapiens
TIAQDYGVLK

SEQ ID NO: 522 - protein, 9 aa, Homo sapiens
IGHPAPNFK

SEQ ID NO: 523 - protein, 10 aa, Homo sapiens
LVQAFQFTDK

SEQ ID NO: 524 - protein, 14 aa, Homo sapiens
DYGVYLEDSGHTLR

SEQ ID NO: 525 - protein, 13 aa, Homo sapiens
IPLLSDLTHQISK

SEQ ID NO: 526 - protein, 12 aa, Homo sapiens
VSVADHSLHLSK

SEQ ID NO: 527 - protein, 10 aa, Homo sapiens
LVQAFQYTDK

SEQ ID NO: 528 - protein, 11 aa, Homo sapiens
QITLNDLPVGR

SEQ ID NO: 529 - protein, 19 aa, Homo sapiens
ISKPAPYWEGTAVIDGEFK

SEQ ID NO: 530 - protein, 8 aa, Homo sapiens
QGGLGPIR

SEQ ID NO: 531 - protein, 14 aa, Homo sapiens
STGGAPTFNVTVTK

SEQ ID NO: 532 - protein, 8 aa, Homo sapiens
TLVLLMGK

SEQ ID NO: 533 - protein, 12 aa, Homo sapiens
DSPSVWAAVPGK

SEQ ID NO: 534 - protein, 16 aa, Homo sapiens
TFVNITPAEVGVLVGK

SEQ ID NO: 535 - protein, 14 aa, Homo sapiens
SSFYVNGLTLGGQK

SEQ ID NO: 536 - protein, 14 aa, Homo sapiens
DSLLQDGEFSMDLR

SEQ ID NO: 537 - protein, 17 aa, Homo sapiens
AQGFTEDTIVFLPQTDK

SEQ ID NO: 538 - protein, 19 aa, Homo sapiens
SVVAPATDGGLNLTSTFLR

SEQ ID NO: 539 - protein, 14 aa, Homo sapiens
WFSAGLASNSSWLR

SEQ ID NO: 540 - protein, 16 aa, Homo sapiens
TMLLQPAGSLGSYSYR

SEQ ID NO: 541 - protein, 10 aa, Homo sapiens
ALAAVLEELR

SEQ ID NO: 542 - protein, 13 aa, Homo sapiens
LTSALDELLQATR

SEQ ID NO: 543 - protein, 11 aa, Homo sapiens
ETGGAESCHIR

SEQ ID NO: 544 - protein, 9 aa, Homo sapiens
TILFSYGTK

SEQ ID NO: 545 - protein, 9 aa, Homo sapiens
AHAWPSPYK

SEQ ID NO: 546 - protein, 13 aa, Homo sapiens
TNVNVFSELSAPR

SEQ ID NO: 547 - protein, 7 aa, Homo sapiens
SYGVENR

SEQ ID NO: 548 - protein, 35 aa, Homo sapiens
AYSQEEITQGFEETGDTLYAPYSTHFQLQNQPPQK

SEQ ID NO: 549 - protein, 10 aa, Homo sapiens
MATTVPDGCR

SEQ ID NO: 550 - protein, 24 aa, Homo sapiens
FFLFGILFSICFSCLLAHAVSLTK

SEQ ID NO: 551 - protein, 8 aa, Homo sapiens
QVSVEEAK

SEQ ID NO: 552 - protein, 7 aa, Homo sapiens
SDLEDKR

SEQ ID NO: 553 - protein, 9 aa, Homo sapiens
VPVILVGNK

SEQ ID NO: 554 - protein, 7 aa, Homo sapiens
VDLESER

SEQ ID NO: 555 - protein, 12 aa, Homo sapiens
YEKVPVILVGNK

SEQ ID NO: 556 - protein, 12 aa, Homo sapiens
ASVDELFAEIVR

SEQ ID NO: 557 - protein, 15 aa, Homo sapiens
SALTVQFVTGSFIEK

SEQ ID NO: 558 - protein, 8 aa, Homo sapiens
EVSYGEGK

SEQ ID NO: 559 - protein, 7 aa, Homo sapiens
QAHELAK

SEQ ID NO: 560 - protein, 15 aa, Homo sapiens
TGEGFLCVFAINNSK

SEQ ID NO: 561 - protein, 15 aa, Homo sapiens
AISSIGLECQSVTSR

SEQ ID NO: 562 - protein, 8 aa, Homo sapiens
GDLATCPR

SEQ ID NO: 563 - protein, 12 aa, Homo sapiens
TLCSMEEAINER

SEQ ID NO: 564 - protein, 18 aa, Homo sapiens
AETTCHCQCAGMDWTGAR

SEQ ID NO: 565 - protein, 7 aa, Homo sapiens
ELTIGSK

SEQ ID NO: 566 - protein, 18 aa, Homo sapiens
MACPLDQAIGLLVAIFHK

SEQ ID NO: 567 - protein, 15 aa, Homo sapiens
VIEHIMEDLDTNADK

SEQ ID NO: 568 - protein, 8 aa, Homo sapiens
LTWASHEK

SEQ ID NO: 569 - protein, 13 aa, Homo sapiens
QLSFEEFIMLMAR

SEQ ID NO: 570 - protein, 15 aa, Homo sapiens
NIETIINTFHQYSVK

SEQ ID NO: 571 - protein, 14 aa, Homo sapiens
GDGPVQGIINFEQK

SEQ ID NO: 572 - protein, 12 aa, Homo sapiens
HVGDLGNVTADK

SEQ ID NO: 573 - protein, 10 aa, Homo sapiens
LACGVIGIAQ

SEQ ID NO: 574 - protein, 24 aa, Homo sapiens
DGVADVSIEDSVISLSGDHCIIGR

SEQ ID NO: 575 - protein, 10 aa, Homo sapiens
ASNLLLGFDR

SEQ ID NO: 576 - protein, 11 aa, Homo sapiens
NLLVNTLYTVR

SEQ ID NO: 577 - protein, 10 aa, Homo sapiens
YSTNEGETWK

SEQ ID NO: 578 - protein, 8 aa, Homo sapiens
NLQLSLPR

SEQ ID NO: 579 - protein, 9 aa, Homo sapiens
NVLVTLYER

SEQ ID NO: 580 - protein, 16 aa, Homo sapiens
YIPPCLDSELTEFPLR

SEQ ID NO: 581 - protein, 13 aa, Homo sapiens
LEAGDHPVELLAR

SEQ ID NO: 582 - protein, 10 aa, Homo sapiens
LHLDYIGPCK

SEQ ID NO: 583 - protein, 20 aa, Homo sapiens
EQANAVSEAVVSSVNTVATK

SEQ ID NO: 584 - protein, 16 aa, Homo sapiens
TVEEAENIAVTSGVVR

SEQ ID NO: 585 - protein, 13 aa, Homo sapiens
ENVVQSVTSVAEK

SEQ ID NO: 586 - protein, 9 aa, Homo sapiens
EGVVGAVEK

SEQ ID NO: 587 - protein, 12 aa, Homo sapiens
EEVAEEAQSGGD

SEQ ID NO: 588 - protein, 9 aa, Homo sapiens
DVDLEFLAK

SEQ ID NO: 589 - protein, 12 aa, Homo sapiens
EVDIGIPDATGR

SEQ ID NO: 590 - protein, 13 aa, Homo sapiens
LDQLIYIPLPDEK

SEQ ID NO: 591 - protein, 9 aa, Homo sapiens
LEILQIHTK

SEQ ID NO: 592 - protein, 15 aa, Homo sapiens
DNTLQVDINGFTTGR

SEQ ID NO: 593 - protein, 10 aa, Homo sapiens
VEQHVELYQK

SEQ ID NO: 594 - protein, 8 aa, Homo sapiens
GGEIEGFR

SEQ ID NO: 595 - protein, 19 aa, Homo sapiens
VAGESAEPEPEPEADYYAK

SEQ ID NO: 596 - protein, 11 aa, Homo sapiens
EAVPEPVLLSR

SEQ ID NO: 597 - protein, 8 aa, Homo sapiens
IELPTTVK

SEQ ID NO: 598 - protein, 13 aa, Homo sapiens
DLSLISPLAQAVR

SEQ ID NO: 599 - protein, 8 aa, Homo sapiens
IAVSYQTK

SEQ ID NO: 600 - protein, 12 aa, Homo sapiens
ANALLANGVELR

SEQ ID NO: 601 - protein, 21 aa, Homo sapiens
DNQLVVPSEGLYLIYSQVLFK

SEQ ID NO: 602 - protein, 8 aa, Homo sapiens
EVVLQHVR

SEQ ID NO: 603 - protein, 20 aa, Homo sapiens
SSVAADVISLLLNGDGGVGR

SEQ ID NO: 604 - protein, 14 aa, Homo sapiens
CQCPAGAALQADGR

SEQ ID NO: 605 - protein, 7 aa, Homo sapiens
GHLMTVR

SEQ ID NO: 606 - protein, 15 aa, Homo sapiens
LWIGLQLPPGCGDPK

SEQ ID NO: 607 - protein, 15 aa, Homo sapiens
GFQWVTGDNNTSYSR

SEQ ID NO: 608 - protein, 8 aa, Homo sapiens
YLGEEYVK

SEQ ID NO: 609 - protein, 8 aa, Homo sapiens
DSAHGFLK

SEQ ID NO: 610 - protein, 12 aa, Homo sapiens
FVFGTTPEDILR

SEQ ID NO: 611 - protein, 17 aa, Homo sapiens
QHVVSVEEALLATGQWK

SEQ ID NO: 612 - protein, 12 aa, Homo sapiens
GTSQNDPNWVVR

SEQ ID NO: 613 - protein, 10 aa, Homo sapiens
SITLFVQEDR

SEQ ID NO: 614 - protein, 13 aa, Homo sapiens
LTFDSSFSPNTGK

SEQ ID NO: 615 - protein, 20 aa, Homo sapiens
VNNSSLIGLGYTQTLKPGIK

SEQ ID NO: 616 - protein, 10 aa, Homo sapiens
LTLSALLDGK

SEQ ID NO: 617 - protein, 11 aa, Homo sapiens
VTQSNFAVGYK

SEQ ID NO: 618 - protein, 12 aa, Homo sapiens
YQIDPDACFSAK

SEQ ID NO: 619 - protein, 8 aa, Homo sapiens
EDIFYTSK

SEQ ID NO: 620 - protein, 8 aa, Homo sapiens
LAIEAGFR

SEQ ID NO: 621 - protein, 6 aa, Homo sapiens
NFDIPK

SEQ ID NO: 622 - protein, 20 aa, Homo sapiens
SALTLQFMYDEFVEDYEPTK

SEQ ID NO: 623 - protein, 11 aa, Homo sapiens
VIMVGSGGVGK

SEQ ID NO: 624 - protein, 15 aa, Homo sapiens
SALTVQFVTGTFIEK

SEQ ID NO: 625 - protein, 12 aa, Homo sapiens
QGVEDAFYTLVR

SEQ ID NO: 626 - protein, 10 aa, Homo sapiens
AGEVQEPELR

SEQ ID NO: 627 - protein, 7 aa, Homo sapiens
IDVHWTR

SEQ ID NO: 628 - protein, 12 aa, Homo sapiens
GKVEEVELPVEK

SEQ ID NO: 629 - protein, 13 aa, Homo sapiens
FSGSGSGTDFTLK

SEQ ID NO: 630 - protein, 9 aa, Homo sapiens
GDFCIQVGR

SEQ ID NO: 631 - protein, 12 aa, Homo sapiens
TFIAIKPDGVQR

SEQ ID NO: 632 - protein, 17 aa, Homo sapiens
VMLGETNPADSKPGTIR

SEQ ID NO: 633 - protein, 11 aa, Homo sapiens
LVVVGAGGVGK

SEQ ID NO: 634 - protein, 7 aa, Homo sapiens
QAQDLAR

SEQ ID NO: 635 - protein, 12 aa, Homo sapiens
SYGIPFIETSAK

SEQ ID NO: 636 - protein, 15 aa, Homo sapiens
TGEGFLCVFAINNTK

SEQ ID NO: 637 - protein, 14 aa, Homo sapiens
ITPNLAEFAFSLYR

SEQ ID NO: 638 - protein, 15 aa, Homo sapiens
LQHLENELTHDIITK

SEQ ID NO: 639 - protein, 10 aa, Homo sapiens
LSITGTYDLK

SEQ ID NO: 640 - protein, 18 aa, Homo sapiens
LYHSEAFTVNFGDTEEAK

SEQ ID NO: 641 - protein, 10 aa, Homo sapiens
SVLGQLGITK

SEQ ID NO: 642 - protein, 11 aa, Homo sapiens
ATWSGAVLAGR

SEQ ID NO: 643 - protein, 20 aa, Homo sapiens
DGVSEGQFQQVLHHELLAIR

SEQ ID NO: 644 - protein, 13 aa, Homo sapiens
DYQPGITFIVVQK

SEQ ID NO: 645 - protein, 11 aa, Homo sapiens
SASFNTDPYVR

SEQ ID NO: 646 - protein, 7 aa, Homo sapiens
SFTEQLR

SEQ ID NO: 647 - protein, 12 aa, Homo sapiens
VELEVTLPGEGK

SEQ ID NO: 648 - protein, 12 aa, Homo sapiens
VLQPPSILYGGR

SEQ ID NO: 649 - protein, 11 aa, Homo sapiens
AGLILFGNDDK

SEQ ID NO: 650 - protein, 15 aa, Homo sapiens
ANATEFGLASGVFTR

SEQ ID NO: 651 - protein, 12 aa, Homo sapiens
DLGEAALNEYLR

SEQ ID NO: 652 - protein, 12 aa, Homo sapiens
FADGDLDAVLSR

SEQ ID NO: 653 - protein, 21 aa, Homo sapiens
GAASSVLELTEAELVTAEAVR

SEQ ID NO: 654 - protein, 16 aa, Homo sapiens
GVVNVLPGSGSLVGQR

SEQ ID NO: 655 - protein, 12 aa, Homo sapiens
VLEVEDSTDFFK

SEQ ID NO: 656 - protein, 12 aa, Homo sapiens
ADDGRPFPQVIK

SEQ ID NO: 657 - protein, 8 aa, Homo sapiens
ALQASALK

SEQ ID NO: 658 - protein, 8 aa, Homo sapiens
ELSDIAHR

SEQ ID NO: 659 - protein, 14 aa, Homo sapiens
GILAADESTGSIAK

SEQ ID NO: 660 - protein, 20 aa, Homo sapiens
IGEHTPSALAIMENANVLAR

SEQ ID NO: 661 - protein, 9 aa, Homo sapiens
QLLLTADDR

SEQ ID NO: 662 - protein, 12 aa, Homo sapiens
DAPLEYDDSVQR

SEQ ID NO: 663 - protein, 9 aa, Homo sapiens
HIIQLQSIK

SEQ ID NO: 664 - protein, 13 aa, Homo sapiens
IVTATVNNSVLQK

SEQ ID NO: 665 - protein, 11 aa, Homo sapiens
QILDQTSEINK

SEQ ID NO: 666 - protein, 10 aa, Homo sapiens
QNSIIEELEK

SEQ ID NO: 667 - protein, 21 aa, Homo sapiens
SGHTTNGIYTLTFPNSTEEIK

SEQ ID NO: 668 - protein, 11 aa, Homo sapiens
ATLYVTAIEDR

SEQ ID NO: 669 - protein, 14 aa, Homo sapiens
DKWLAPDGLIFPDR

SEQ ID NO: 670 - protein, 10 aa, Homo sapiens
EPLVDVVDPK

SEQ ID NO: 671 - protein, 9 aa, Homo sapiens
LDHVVTIIK

SEQ ID NO: 672 - protein, 17 aa, Homo sapiens
NDYVHALVAYFNIEFTR

SEQ ID NO: 673 - protein, 15 aa, Homo sapiens
TGFSTSPESPYTHWK

SEQ ID NO: 674 - protein, 9 aa, Homo sapiens
ALYVHGGYK

SEQ ID NO: 675 - protein, 16 aa, Homo sapiens
EQYAVVGHSAHIVTLK

SEQ ID NO: 676 - protein, 12 aa, Homo sapiens
IDSTGNVTNELR

SEQ ID NO: 677 - protein, 7 aa, Homo sapiens
LADDLYR

SEQ ID NO: 678 - protein, 10 aa, Homo sapiens
LTLTPWVGLR

SEQ ID NO: 679 - protein, 8 aa, Homo sapiens
SVNNVVVR

SEQ ID NO: 680 - protein, 9 aa, Homo sapiens
YGHSLALYK

SEQ ID NO: 681 - protein, 7 aa, Homo sapiens
EFEETAK

SEQ ID NO: 682 - protein, 16 aa, Homo sapiens
ELEGWEPDDDPIEEHK

SEQ ID NO: 683 - protein, 15 aa, Homo sapiens
MGAPTLPPAWQPFLK

SEQ ID NO: 684 - protein, 14 aa, Homo sapiens
NWPFLEGCACTPER

SEQ ID NO: 685 - protein, 12 aa, Homo sapiens
QFEELTLGEFLK

SEQ ID NO: 686 - protein, 11 aa, Homo sapiens
DIQGSLQDIFK

SEQ ID NO: 687 - protein, 12 aa, Homo sapiens
INENTGSVSVTR

SEQ ID NO: 688 - protein, 7 aa, Homo sapiens
TLFVHAR

SEQ ID NO: 689 - protein, 11 aa, Homo sapiens
VNSDGGLVALR

SEQ ID NO: 690 - protein, 9 aa, Homo sapiens
YEVSSPYFK

SEQ ID NO: 691 - protein, 7 aa, Homo sapiens
FTQDTFR

SEQ ID NO: 692 - protein, 22 aa, Homo sapiens
IFYSITGPGADSPPEGVFAVEK

SEQ ID NO: 693 - protein, 15 aa, Homo sapiens
LTVTDLDAPNSPAWR

SEQ ID NO: 694 - protein, 14 aa, Homo sapiens
STGTISVISSGLDR

SEQ ID NO: 695 - protein, 16 aa, Homo sapiens
YEAHVPENAVGHEVQR

SEQ ID NO: 696 - protein, 9 aa, Homo sapiens
AASQPGELK

SEQ ID NO: 697 - protein, 8 aa, Homo sapiens
LLIPGNYK

SEQ ID NO: 698 - protein, 13 aa, Homo sapiens
LQQEDGISFEYHR

SEQ ID NO: 699 - protein, 7 aa, Homo sapiens
NFPDLDR

SEQ ID NO: 700 - protein, 12 aa, Homo sapiens
NSLISYLEQIHR

SEQ ID NO: 701 - protein, 10 aa, Homo sapiens
SNAQGIDLNR

SEQ ID NO: 702 - protein, 13 aa, Homo sapiens
YIGNMHGNEAVGR

SEQ ID NO: 703 - protein, 10 aa, Homo sapiens
ALSIGFETCR

SEQ ID NO: 704 - protein, 7 aa, Homo sapiens
EQWFGNR

SEQ ID NO: 705 - protein, 9 aa, Homo sapiens
FAGVFHVEK

SEQ ID NO: 706 - protein, 8 aa, Homo sapiens
NLQNVDMK

SEQ ID NO: 707 - protein, 8 aa, Homo sapiens
TEAADLCK

SEQ ID NO: 708 - protein, 12 aa, Homo sapiens
YGFIEGHVVIPR

SEQ ID NO: 709 - protein, 12 aa, Homo sapiens
ASSIIDELFQDR

SEQ ID NO: 710 - protein, 11 aa, Homo sapiens
ELDESLQVAER

SEQ ID NO: 711 - protein, 9 aa, Homo sapiens
IDSLLENDR

SEQ ID NO: 712 - protein, 17 aa, Homo sapiens
LFDSDPITVTVPVEVSR

SEQ ID NO: 713 - protein, 11 aa, Homo sapiens
AQCGGGLLGVR

SEQ ID NO: 714 - protein, 8 aa, Homo sapiens
ITEEFLGK

SEQ ID NO: 715 - protein, 10 aa, Homo sapiens
LLASDAGLYR

SEQ ID NO: 716 - protein, 19 aa, Homo sapiens
VSVPTHPEAVGDASLTVVK

SEQ ID NO: 717 - protein, 10 aa, Homo sapiens
YTLNFEAAQK

SEQ ID NO: 718 - protein, 19 aa, Homo sapiens
EIYCPAPPQIDNGIIQGER

SEQ ID NO: 719 - protein, 13 aa, Homo sapiens
GSQWSDIEEFCNR

SEQ ID NO: 720 - protein, 8 aa, Homo sapiens
LTCLQNLK

SEQ ID NO: 721 - protein, 9 aa, Homo sapiens
SCPNPGEIR

SEQ ID NO: 722 - protein, 12 aa, Homo sapiens
TSFPEDTVITYK

SEQ ID NO: 723 - protein, 10 aa, Homo sapiens
TTTPNAQATR

SEQ ID NO: 724 - protein, 24 aa, Homo sapiens
VPPTVQKPTTVNVPTTEVSPTSQK

SEQ ID NO: 725 - protein, 11 aa, Homo sapiens
IESSSLQGLGR

SEQ ID NO: 726 - protein, 8 aa, Homo sapiens
IYWVDLER

SEQ ID NO: 727 - protein, 8 aa, Homo sapiens
LFWIQYNR

SEQ ID NO: 728 - protein, 11 aa, Homo sapiens
NQVTPLDILSK

SEQ ID NO: 729 - protein, 14 aa, Homo sapiens
FSFLLHFYTVPIPK

SEQ ID NO: 730 - protein, 12 aa, Homo sapiens
GEVTYTTSQVSK

SEQ ID NO: 731 - protein, 18 aa, Homo sapiens
GPITSAAELNDPQSILLR

SEQ ID NO: 732 - protein, 13 aa, Homo sapiens
LPDTPQGLLGEAR

SEQ ID NO: 733 - protein, 10 aa, Homo sapiens
TGSQDQEVHR

SEQ ID NO: 734 - protein, 10 aa, Homo sapiens
TQILEWAAER

SEQ ID NO: 735 - protein, 10 aa, Homo sapiens
VLPGHSAGPR

SEQ ID NO: 736 - protein, 10 aa, Homo sapiens
AAGEGLLTLR

SEQ ID NO: 737 - protein, 16 aa, Homo sapiens
APEPQLSPGSDASEVR

SEQ ID NO: 738 - protein, 14 aa, Homo sapiens
VSPDHVTLLDPASK

SEQ ID NO: 739 - protein, 9 aa, Homo sapiens
VYSQVTVQR

SEQ ID NO: 740 - protein, 8 aa, Homo sapiens
YAFSLLAR

SEQ ID NO: 741 - protein, 8 aa, Homo sapiens
ILYDFTAR

SEQ ID NO: 742 - protein, 18 aa, Homo sapiens
SQPVSQPLTYESGPDEVR

SEQ ID NO: 743 - protein, 14 aa, Homo sapiens
LLGEVDHYQLALGK

SEQ ID NO: 744 - protein, 9 aa, Homo sapiens
QDGSVDFFR

SEQ ID NO: 745 - protein, 9 aa, Homo sapiens
TFAHYATFR

SEQ ID NO: 746 - protein, 10 aa, Homo sapiens
YAVSEAAAHK

SEQ ID NO: 747 - protein, 9 aa, Homo sapiens
YGIDWASGR

SEQ ID NO: 748 - protein, 17 aa, Homo sapiens
ASTPNGYDNGIIWATWK

SEQ ID NO: 749 - protein, 15 aa, Homo sapiens
IHLISTQSAIPYALR

SEQ ID NO: 750 - protein, 11 aa, Homo sapiens
QSGLYFIKPLK

SEQ ID NO: 751 - protein, 10 aa, Homo sapiens
TSTADYAMFK

SEQ ID NO: 752 - protein, 13 aa, Homo sapiens
YEASILTHDSSIR

SEQ ID NO: 753 - protein, 13 aa, Homo sapiens
AGALNSNDAFVLK

SEQ ID NO: 754 - protein, 15 aa, Homo sapiens
EVQGFESATFLGYFK

SEQ ID NO: 755 - protein, 17 aa, Homo sapiens
QTQVSVLPEGGETPLFK

SEQ ID NO: 756 - protein, 8 aa, Homo sapiens
TGAQELLR

SEQ ID NO: 757 - protein, 9 aa, Homo sapiens
YIETDPANR

SEQ ID NO: 758 - protein, 13 aa, Homo sapiens
GEGEPCGGGGAGR

SEQ ID NO: 759 - protein, 14 aa, Homo sapiens
GTCEQGPSIVTPPK

SEQ ID NO: 760 - protein, 8 aa, Homo sapiens
TELLPGDR

SEQ ID NO: 761 - protein, 15 aa, Homo sapiens
DVSTPPTVLPDNFPR

SEQ ID NO: 762 - protein, 8 aa, Homo sapiens
FFQYDTWK

SEQ ID NO: 763 - protein, 10 aa, Homo sapiens
GFYFSRPASR

SEQ ID NO: 764 - protein, 9 aa, Homo sapiens
GIVEECCFR

SEQ ID NO: 765 - protein, 16 aa, Homo sapiens
SCDLALLETYCATPAK

SEQ ID NO: 766 - protein, 9 aa, Homo sapiens
DFWLHANNK

SEQ ID NO: 767 - protein, 8 aa, Homo sapiens
DNHLALIK

SEQ ID NO: 768 - protein, 8 aa, Homo sapiens
EHSVELHK

SEQ ID NO: 769 - protein, 10 aa, Homo sapiens
TDPGVFIGVK

SEQ ID NO: 770 - protein, 22 aa, Homo sapiens
VLLSYYESQHPSNESGDGVDGK

SEQ ID NO: 771 - protein, 17 aa, Homo sapiens
LKPEDITQIQPQQLVLR

SEQ ID NO: 772 - protein, 11 aa, Homo sapiens
FCECDNFNCDR

SEQ ID NO: 773 - protein, 17 aa, Homo sapiens
LLVFSTDAGFHFAGDGK

SEQ ID NO: 774 - protein, 10 aa, Homo sapiens
LSEGVTISYK

SEQ ID NO: 775 - protein, 21 aa, Homo sapiens
LSENNIQTIFAVTEEFQPVYK

SEQ ID NO: 776 - protein, 9 aa, Homo sapiens
FAHTVVTSR

SEQ ID NO: 777 - protein, 12 aa, Homo sapiens
GPDVLTATVSGK

SEQ ID NO: 778 - protein, 9 aa, Homo sapiens
LGVYELLLK

SEQ ID NO: 779 - protein, 16 aa, Homo sapiens
SPEQQETVLDGNLIIR

SEQ ID NO: 780 - protein, 21 aa, Homo sapiens
AVCGGVLVHPQWVLTAAHCIR

SEQ ID NO: 781 - protein, 16 aa, Homo sapiens
FLRPGDDSSHDLMLLR

SEQ ID NO: 782 - protein, 12 aa, Homo sapiens
HSQPWQVLVASR

SEQ ID NO: 783 - protein, 12 aa, Homo sapiens
LSEPAELTDAVK

SEQ ID NO: 784 - protein, 7 aa, Homo sapiens
SVILLGR

SEQ ID NO: 785 - protein, 19 aa, Homo sapiens
DIPTNSPELEETLTHTITK

SEQ ID NO: 786 - protein, 12 aa, Homo sapiens
LNAENNATFYFK

SEQ ID NO: 787 - protein, 9 aa, Homo sapiens
QVVAGLNFR

SEQ ID NO: 788 - protein, 11 aa, Homo sapiens
TVGSDTFYSFK

SEQ ID NO: 789 - protein, 8 aa, Homo sapiens
YFIDFVAR

SEQ ID NO: 790 - protein, 15 aa, Homo sapiens
YNSQNQSNNQFVLYR

SEQ ID NO: 791 - protein, 11 aa, Homo sapiens
CCSGAIIVLTK

SEQ ID NO: 792 - protein, 18 aa, Homo sapiens
GADFLVTEVENGGSLGSK

SEQ ID NO: 793 - protein, 13 aa, Homo sapiens
IYVDDGLISLQVK

SEQ ID NO: 794 - protein, 22 aa, Homo sapiens
LAPITSDPTEATAVGAVEASFK

SEQ ID NO: 795 - protein, 11 aa, Homo sapiens
LDIDSPPITAR

SEQ ID NO: 796 - protein, 11 aa, Homo sapiens
DAPSWDPVALK

SEQ ID NO: 797 - protein, 13 aa, Homo sapiens
HFVIDGHPVSFSK

SEQ ID NO: 798 - protein, 10 aa, Homo sapiens
LAALSIEEGK

SEQ ID NO: 799 - protein, 8 aa, Homo sapiens
LITEEANR

SEQ ID NO: 800 - protein, 14 aa, Homo sapiens
SGVLSVSSGAAAHR

SEQ ID NO: 801 - protein, 12 aa, Homo sapiens
SLLSDVEELVEK

SEQ ID NO: 802 - protein, 15 aa, Homo sapiens
VFLTVPSLSSTAEEK

SEQ ID NO: 803 - protein, 18 aa, Homo sapiens
EQTVSVSGAFQINTFDLR

SEQ ID NO: 804 - protein, 12 aa, Homo sapiens
GILTVDELLAIR

SEQ ID NO: 805 - protein, 8 aa, Homo sapiens
IPLNDLFR

SEQ ID NO: 806 - protein, 7 aa, Homo sapiens
SHTALLR

SEQ ID NO: 807 - protein, 10 aa, Homo sapiens
VQPFNVTQGK

SEQ ID NO: 808 - protein, 9 aa, Homo sapiens
YLDFVFAVK

SEQ ID NO: 809 - protein, 15 aa, Homo sapiens
DLADELALVDVIEDK

SEQ ID NO: 810 - protein, 8 aa, Homo sapiens
FIIPNVVK

SEQ ID NO: 811 - protein, 9 aa, Homo sapiens
LVIITAGAR

SEQ ID NO: 812 - protein, 10 aa, Homo sapiens
SADTLWGIQK

SEQ ID NO: 813 - protein, 10 aa, Homo sapiens
VTLTSEEEAR

SEQ ID NO: 814 - protein, 10 aa, Homo sapiens
ELAPLFEELR

SEQ ID NO: 815 - protein, 23 aa, Homo sapiens
LPLVVSFIASSSANTGLIVSLEK

SEQ ID NO: 816 - protein, 15 aa, Homo sapiens
LPSVEGLHAIVVSDR

SEQ ID NO: 817 - protein, 16 aa, Homo sapiens
SIICYYNTYQVVQFNR

SEQ ID NO: 818 - protein, 7 aa, Homo sapiens
AGYVLHR

SEQ ID NO: 819 - protein, 15 aa, Homo sapiens
DTFYSLGSSLDITFR

SEQ ID NO: 820 - protein, 8 aa, Homo sapiens
WPEPVFGR

SEQ ID NO: 821 - protein, 10 aa, Homo sapiens
WTLTAPPGYR

SEQ ID NO: 822 - protein, 15 aa, Homo sapiens
FLNSNSGLQGLQFYR

SEQ ID NO: 823 - protein, 10 aa, Homo sapiens
IGLASALQPR

SEQ ID NO: 824 - protein, 14 aa, Homo sapiens
NDVVFQPISGEDVR

SEQ ID NO: 825 - protein, 12 aa, Homo sapiens
SLEPFTLEILAR

SEQ ID NO: 826 - protein, 22 aa, Homo sapiens
TVDFTSPLFKPATGFPLGSSLR

SEQ ID NO: 827 - protein, 14 aa, Homo sapiens
WNDKPYLCALYQQR

SEQ ID NO: 828 - protein, 14 aa, Homo sapiens
NIIHGSDSVESAEK

SEQ ID NO: 829 - protein, 10 aa, Homo sapiens
ALHIPFPVEK

SEQ ID NO: 830 - protein, 18 aa, Homo sapiens
DEDGKPYSPSEYSLQQTR

SEQ ID NO: 831 - protein, 9 aa, Homo sapiens
DGNVFLVPK

SEQ ID NO: 832 - protein, 12 aa, Homo sapiens
EQFNEAQLALIR

SEQ ID NO: 833 - protein, 15 aa, Homo sapiens
IINLPVVDFNEMMSK

SEQ ID NO: 834 - protein, 15 aa, Homo sapiens
LENIVELEQDLDHLK

SEQ ID NO: 835 - protein, 8 aa, Homo sapiens
AIAVDPIR

SEQ ID NO: 836 - protein, 8 aa, Homo sapiens
DGVVSVNK

SEQ ID NO: 837 - protein, 14 aa, Homo sapiens
EGTSLGEVGGPDLK

SEQ ID NO: 838 - protein, 12 aa, Homo sapiens
ESYNVQLQLPAR

SEQ ID NO: 839 - protein, 12 aa, Homo sapiens
HAQAQYAYPGAR

SEQ ID NO: 840 - protein, 17 aa, Homo sapiens
ITQTAEGLDPENYLSIK

SEQ ID NO: 841 - protein, 11 aa, Homo sapiens
LANPLHFYEAR

SEQ ID NO: 842 - protein, 17 aa, Homo sapiens
AIPVAQDLNAPSDWDSR

SEQ ID NO: 843 - protein, 19 aa, Homo sapiens
ANDESNEHSDVIDSQELSK

SEQ ID NO: 844 - protein, 9 aa, Homo sapiens
GDSVVYGLR

SEQ ID NO: 845 - protein, 19 aa, Homo sapiens
QNLLAPQNAVSSEETNDFK

SEQ ID NO: 846 - protein, 16 aa, Homo sapiens
YPDAVATWLNPDPSQK

SEQ ID NO: 847 - protein, 9 aa, Homo sapiens
ELNEALELK

SEQ ID NO: 848 - protein, 10 aa, Homo sapiens
LGFLHSGTAK

SEQ ID NO: 849 - protein, 19 aa, Homo sapiens
RPILTIITLEDSSGNLLGR

SEQ ID NO: 850 - protein, 9 aa, Homo sapiens
TYQGSYGFR

SEQ ID NO: 851 - protein, 7 aa, Homo sapiens
VEYLDDR

SEQ ID NO: 852 - protein, 8 aa, Homo sapiens
AHGVHATK

SEQ ID NO: 853 - protein, 19 aa, Homo sapiens
LEEHLECACATTSLNPDYR

SEQ ID NO: 854 - protein, 18 aa, Homo sapiens
LLEIDSVGSEDSLDTSLR

SEQ ID NO: 855 - protein, 7 aa, Homo sapiens
SQIHSIR

SEQ ID NO: 856 - protein, 8 aa, Homo sapiens
TVIYEIPR

SEQ ID NO: 857 - protein, 12 aa, Homo sapiens
AGALQLLLVGDK

SEQ ID NO: 858 - protein, 20 aa, Homo sapiens
ATYFGSIVLLSPAVIDSPLK

SEQ ID NO: 859 - protein, 11 aa, Homo sapiens
AVEPQLQEEER

SEQ ID NO: 860 - protein, 12 aa, Homo sapiens
EGHFYYNISEVK

SEQ ID NO: 861 - protein, 15 aa, Homo sapiens
FLEQELETITIPDLR

SEQ ID NO: 862 - protein, 14 aa, Homo sapiens
VYDFLSTFITSGMR

SEQ ID NO: 863 - protein, 8 aa, Homo sapiens
DFIATLGK

SEQ ID NO: 864 - protein, 15 aa, Homo sapiens
ELSELSLLSLYGIHK

SEQ ID NO: 865 - protein, 10 aa, Homo sapiens
FQELESETLK

SEQ ID NO: 866 - protein, 7 aa, Homo sapiens
FVTLVFR

SEQ ID NO: 867 - protein, 12 aa, Homo sapiens
SPIDTFPTDPIK

SEQ ID NO: 868 - protein, 9 aa, Homo sapiens
SFEDIHHYR

SEQ ID NO: 869 - protein, 8 aa, Homo sapiens
EILDAFDK

SEQ ID NO: 870 - protein, 15 aa, Homo sapiens
EIVDSYLPVILDIIK

SEQ ID NO: 871 - protein, 10 aa, Homo sapiens
GSAVWCQNVK

SEQ ID NO: 872 - protein, 7 aa, Homo sapiens
LVGYLDR

SEQ ID NO: 873 - protein, 9 aa, Homo sapiens
QEILAALEK

SEQ ID NO: 874 - protein, 9 aa, Homo sapiens
DGLIPLEIR

SEQ ID NO: 875 - protein, 14 aa, Homo sapiens
GGFVLLDGETFEVK

SEQ ID NO: 876 - protein, 13 aa, Homo sapiens
LTGQLFLGGSIVK

SEQ ID NO: 877 - protein, 10 aa, Homo sapiens
LVLPSLISSR

SEQ ID NO: 878 - protein, 10 aa, Homo sapiens
NEGGTWSVEK

SEQ ID NO: 879 - protein, 8 aa, Homo sapiens
FFESHVAR

SEQ ID NO: 880 - protein, 14 aa, Homo sapiens
ILNTPNCALQIVAR

SEQ ID NO: 881 - protein, 8 aa, Homo sapiens
WIQEYLEK

SEQ ID NO: 882 - protein, 11 aa, Homo sapiens
DRPFVCAPSSK

SEQ ID NO: 883 - protein, 15 aa, Homo sapiens
HDSATDTIDIAPNHR

SEQ ID NO: 884 - protein, 10 aa, Homo sapiens
TIVLQESIGK

SEQ ID NO: 885 - protein, 12 aa, Homo sapiens
TLSQLSQQEGIK

SEQ ID NO: 886 - protein, 16 aa, Homo sapiens
VIHNSMCIAEIDLIPR

SEQ ID NO: 887 - protein, 21 aa, Homo sapiens
VPNEEDPSLDRPFISEGTTLK

SEQ ID NO: 888 - protein, 16 aa, Homo sapiens
DSTIQVVENGESSQGR

SEQ ID NO: 889 - protein, 10 aa, Homo sapiens
DWVSVVTPAR

SEQ ID NO: 890 - protein, 8 aa, Homo sapiens
FVGQGGAR

SEQ ID NO: 891 - protein, 9 aa, Homo sapiens
SGSVIDQSR

SEQ ID NO: 892 - protein, 7 aa, Homo sapiens
TLDEYWR

SEQ ID NO: 893 - protein, 9 aa, Homo sapiens
VLNLGPITR

SEQ ID NO: 894 - protein, 9 aa, Homo sapiens
ELQVYISPK

SEQ ID NO: 895 - protein, 11 aa, Homo sapiens
GIQVEIYSFPK

SEQ ID NO: 896 - protein, 13 aa, Homo sapiens
LHIDEMDSVPTVR

SEQ ID NO: 897 - protein, 11 aa, Homo sapiens
NTVISVNPSTK

SEQ ID NO: 898 - protein, 15 aa, Homo sapiens
SLEVTFTPVIEDIGK

SEQ ID NO: 899 - protein, 10 aa, Homo sapiens
TQIDSPLNGK

SEQ ID NO: 900 - protein, 13 aa, Homo sapiens
EDFTSLSLVLYSR

SEQ ID NO: 901 - protein, 8 aa, Homo sapiens
ELPEHTVK

SEQ ID NO: 902 - protein, 11 aa, Homo sapiens
HLSLLTTLSNR

SEQ ID NO: 903 - protein, 10 aa, Homo sapiens
THLPEVFLSK

SEQ ID NO: 904 - protein, 7 aa, Homo sapiens
YTFELSR

SEQ ID NO: 905 - protein, 13 aa, Homo sapiens
ALGFEDATQALGR

SEQ ID NO: 906 - protein, 12 aa, Homo sapiens
GLDLTEDTYKPR

SEQ ID NO: 907 - protein, 21 aa, Homo sapiens
QQQHLFGSDVTDCSGNFCLFR

SEQ ID NO: 908 - protein, 14 aa, Homo sapiens
QDFDITDISLLEHR

SEQ ID NO: 909 - protein, 20 aa, Homo sapiens
DETHATYSNTLYLADEIIIR

SEQ ID NO: 910 - protein, 10 aa, Homo sapiens
DRPFFAGLVK

SEQ ID NO: 911 - protein, 13 aa, Homo sapiens
AAIPSALDTDSSK

SEQ ID NO: 912 - protein, 23 aa, Homo sapiens
DPDHSEGSTTLLEGYTSHYPHTK

SEQ ID NO: 913 - protein, 22 aa, Homo sapiens
ISHELDSASSEVNSAVTALWGK

SEQ ID NO: 914 - protein, 5 aa, Homo sapiens
ADDGR

SEQ ID NO: 915 - protein, 7 aa, Homo sapiens
PFPQVIK

SEQ ID NO: 916 - protein, 23 aa, Homo sapiens
IRPFFPQQIHLISTQSAIPYALR

SEQ ID NO: 917 - protein, 16 aa, Homo sapiens
LLGNVLVCVLAHHFGK

SEQ ID NO: 918 - protein, 10 aa, Homo sapiens
AQGYSGLSVK

SEQ ID NO: 919 - protein, 9 aa, Homo sapiens
SVSCPLLSR

SEQ ID NO: 920 - protein, 8 aa, Homo sapiens
FGSDDEGR

SEQ ID NO: 921 - protein, 8 aa, Homo sapiens
IPFTFWAR

SEQ ID NO: 922 - protein, 7 aa, Homo sapiens
QLYLQHR

SEQ ID NO: 923 - protein, 13 aa, Homo sapiens
NVFQLEQAFVLSK

SEQ ID NO: 924 - protein, 18 aa, Homo sapiens
NQHTLYVEVTNEAPFVLK

SEQ ID NO: 925 - protein, 11 aa, Homo sapiens
GLEARPEVVLR

SEQ ID NO: 926 - protein, 12 aa, Homo sapiens
AQPDVHFFQGLR

SEQ ID NO: 927 - protein, 16 aa, Homo sapiens
LSLLEELSLAENQLLK

SEQ ID NO: 928 - protein, 8 aa, Homo sapiens
YSVADIER

SEQ ID NO: 929 - protein, 11 aa, Homo sapiens
VVVLGSGGVGK

SEQ ID NO: 930 - protein, 10 aa, Homo sapiens
YGDLVDYLHR

SEQ ID NO: 931 - protein, 13 aa, Homo sapiens
GGPVQVLEDEELK

SEQ ID NO: 932 - protein, 7 aa, Homo sapiens
TLVVHEK

SEQ ID NO: 933 - protein, 12 aa, Homo sapiens
TFDSSCHFFATK

SEQ ID NO: 934 - protein, 7 aa, Homo sapiens
YSNNSWR

SEQ ID NO: 935 - protein, 4 aa, Artificial Sequence
  Start peptide
MAGR

SEQ ID NO: 936 - protein, 8 aa, Artificial Sequence
  Tag peptide
WSHPQFEK

SEQ ID NO: 937 - protein, 14 aa, Artificial Sequence [sequence omitted]

SEQ ID NO: 938 - protein, 13 aa, Artificial Sequence
  GluFib 2 peptide
GVNDNEEGFFSAR

SEQ ID NO: 939 - protein, 12 aa, Artificial Sequence
  Tag 2 peptide
LAAALEHHHHHH

SEQ ID NO: 940 - protein, 9 aa, Artificial Sequence
  Start/Tag peptide
MWSHPQFEK

SEQ ID NO: 941 - protein, 629 aa, Artificial Sequence
  QconCAT no. 1
MAGRWSHPQFEKEGVNDNEEGFFSARDIVLVAHSALGTQRHIDSAYLYNNEEQVGLAIRELEGWEPDDDPIEEHKQFEELTLGEFLKLVDQNIFSFYLSRVSTLPAITLKYSQAVPAVTEGPIPEVLKVFQEPLFYEAPRAVATVGPISVAIDAGHESFLFYKYSVANDTGFVDIPKAGLQVYNKFEHCNFNDVTTRTSFPEDTVITYKTTTPNAQATRVPPTVQKPTTVNVPTTEVSPTSQKLLDIESQEELEDFPLPTVQRLAINLLAKSQPVSQPLTYESGPDEVREVGVGFATRNTEISFILGQEFDEVTADDRSTITLDGGVLVHVQKTAFYLAEFFVNEARYPVYGVQWHPEKAPAVAEENPKHLDSVLQQLQTEVYRHEVTGWVLVSPLSKITVVDALHEIPVKLKPEDITQIQPQQLVLRLLVFSTDAGFHFAGDGKLGVYELLLKSPEQQETVLDGNLIIRLNAENNATFYFKTVGSDTFYSFKALGFEDATQALGRGLDLTEDTYKPRLADGGATNQGRQQQHLFGSDVTDCSGNFCLFRDGAGDVAFVKQDFDITDISLLEHRDETHATYSNTLYLADEIIIRDWVSVVTPARGVNDNEEGFFSARLAAALEHHHHHH

SEQ ID NO: 942 - protein, 689 aa, Artificial Sequence
  QconCAT no. 2
MAGRWSHPQFEKEGVNDNEEGFFSARYFIDFVARYNSQNQSNNQFVLYRAGQSPQLLIYTLSYRLEIPYTFGQGTKGHTLTLNFTRALQATVGNSYKFFLQGIQLNTILPDARGELFWDDGESLEVLERWGYSSTAITRSLEPFTLEILARIGLASALQPRDRPFFAGLVKNIIHGSDSVESAEKAIPVAQDLNAPSDWDSRANDESNEHSDVIDSQELSKYPDAVATWLNPDPSQKIPLLSDLTHQISKVSVADHSLHLSKAQGFTEDTIVFLPQTDKWFSAGLASNSSWLRAHAWPSPYKTNVNVFSELSAPRAEQWNVNYVETSAKEDENVPFLLVGNKIQEVAGSLIFREIVDSYLPVILDIIKQEILAALEKFFESHVARWIQEYLEKTVEEAENIAVTSGVVREQANAVSEAVVSSVNTVATKELQELVQYPVEHPDKLIVDEAINEDNSVVSLSQPKIELPTTVKTIVLQESIGKEVVLQHVRSSVAADVISLLLNGDGGVGRTIVTTLQDSIRGGVNDNFQGVLQNVRLTFDSSFSPNTGKVNNSSLIGLGYTQTLKPGIKAAIPSALDTDSSKSDLAVPSELALLKFAGVFHVEKDPDHSEGSTTLLEGYTSHYPHTKYGFIEGHVVIPRLLQVVYLHSNNITKIQAIELEDLLRGVNDNEEGFFSARLAAALEHHHHHH

SEQ ID NO: 943 - protein, 799 aa, Artificial Sequence
  QconCAT no. 3
MAGRWSHPQFEKEGVNDNEEGFFSARFNWYVDGVEVHNAKGPSVFPLAPSSKTTPPVLDSDGSFFLYSKQLSFEEFIMLMARLTWASHEKVIEHIMEDLDTNADKLVLPSLISSRAADLLLHSKTNVYISSSAGARITTVSLSAPDALKEDFTSLSLVLYSRYTFELSRTHLPEVFLSKEATDVIIIHSKSIQLPTTVRFSTEYELQQLEQFKALYLQYTDETFRGAYPLSIEPIGVRNNEGTYYSPNYNPQSRGIPGPVGAAGATGARGEPGNIGFPGPKVLEDNSALDKLGTFEVEDQIEAARWEYYDSVYTERTLVLLMGKSTGGAPTFNVTVTKVAAGAFQGLRGQTLLAVAKDLLLPQPDLRIDSLLENDRELDESLQVAERASSIIDELFQDRSLSQQIENIRGANGAPGIAGAPGFPGARFVTDGSVTASGFREQLANPIVSSGNSLFLRDFVEILDGGHEDAPLRIESSSLQGLGRNQVTPLDILSKIYWVDLERQDGSVDFFRYGIDWASGRFADGDLDAVLSRAGLILFGNDDKDLGEAALNEYLRLGVYELLLKSPEQQETVLDGNLIIRFAHTVVTSRYSSDYFQAPSDYRIDITLSSVKELSEALGQIFDSQRFQTFEGDLKQSTLVLFPGDLRLGLGADVAQVTGALRAAYEDFNVQLRAVTLSLDGGDTAIRYPDAVATWLNPDPSQKAIPVAQDLNAPSDWDSRISHELDSASSEVNSAVTALWGKVNVDEVGGEALGRFFESFGDLSTPDAVMGNPKGVNDNEEGFFSARLAAALEHHHHHH

SEQ ID NO: 944 - protein, 792 aa, Artificial Sequence
  QconCAT no. 4
MAGRWSHPQFEKEGVNDNEEGFFSARSDVMYTDWKNWGLSFYADKPETTKEHVAHLLFLRLQHLENELTHDIITKSVLGQLGITKITPNLAEFAFSLYRQGIPFFGQVRNEDSLVFVQTDKLVHVEEPHTETVRDADPDTFFAKFTFEYSRIAPQLSTEELVSLGEKGILAADESTGSIAKADDGRPFPQVIKVSFLSALEEYTKATEHLSTLSEKVQPYLDDFQKLGEVNTYAGDLQKSLAPYAQDTQEKSELTQQLNALFQDKLGPLVEQGRSELEEQLTPVAEETRAFDSDGDGRYSFLELRHDLGHFMLRSNLDEDIIAEENIVSRIHWESASLLRTIYTPGSTVLYRTYFPHFDLSHGSAQVKVGAHAGEYGAEALERMFLSFPTTKGDGPVQGIINFEQKLMEDLDRLQDAEIARDNENVVNEYSSELEKHQLYIDETVNSNIPTNLRIRPFFPQQIHLISTQSAIPYALRYEASILTHDSSIRQSGLYFIKPLKTEVNVLPGAKIQPSGGTNINEALLRFYNQVSTPLLRIYVDDGLISLQVKLDIDSPPITARGADFLVTEVENGGSLGSKSADTLWGIQKVTLTSEEEARDLADELALVDVIEDKSVDPDSPAEASGLRQGGLGPMNIPLVSDPKATAVMPDGQFKDISLSDYKSLEVTFTPVIEDIGKELQVYISPKAGALNSNDAFVLKQTQVSVLPEGGETPLFKYIETDPANRDFADIPNLRLSLEIEQLELQREDVYVVGTVLRGYILVGQAKGVNDNEEGFFSARLAAALEHHHHHH

SEQ ID NO: 945 - protein, 833 aa, Artificial Sequence
  QconCAT no. 5
MWSHPQFEKEGVNDNEEGFFSARSASDLTWDNLKLLGNVLVCVLAHHFGKGEVTYTTSQVSKYSLTYIYTGLSKHINPVAASLIQKLSITGTYDLKSSGPGGQNVNKEGHFYYNISEVKILGATIENSREIPAWVPFDPAAQITKSFEDIHHYRAQGYSGLSVKGLQTSQDARQIDNPDYKIVTATVNNSVLQKDYQPGITFIVVQKHAQAQYAYPGARNHLVEIPPNLPSSLVELRLDHVVTIIKATWSGAVLAGRTGFSTSPESPYTHWKGTFATLSELHCDKLPDTPQGLLGEARDAPSWDPVALKLGELILTSESSRGPDVLTATVSGKEALAENNLNLPKGDDLSTAILKLILYNDGDSLQYIERSVVAPATDGGLNLTSTFLRVELEVTLPGEGKEQYAVVGHSAHIVTLKDVSTPPTVLPDNFPRSVSCPLLSRDGVVSVNKADGVPVYLKVEDAFYTLVREFTPPVQAAYQKVPVILVGNKFGSDDEGRTQILEWAAERATYFGSIVLLSPAVIDSPLKIPFTFWARTELLPGDRFFNVLTTNTDGKAGALQLLLVGDKGAYTQVIFLARGLPDQMLYREFLQSSLRHDSATDTIDIAPNHRLYHSEAFTVNFGDTEEAKQILDQTSEINKLGNLFLNEDLEVKDSTIQVVENGESSQGRDYGVYLEDSGHTLRQVMNGFQNRLTSDSTVYDYAGKTHLAPYSDELRLITEEANREGYYGYTGAFRDYVSQFEGSALGKATLYVTAIEDRGQNSLALHKESYNVQLQLPARWEAEPVYVQRFESSEEQARAKPALEDLRSGVLSVSSGAAAHRLAAALEHHHHHH